European Patent Specification EP 3 548 039 B1, published July 19, 2023. Title: METHODS FOR TREATING DISEASES RELATED TO MITOCHONDRIAL STRESS. Applicant: ALAVI KHORASSANI MOGHADAM, MARCEL VICTOR. Application PCT/US2017/064195. The sequence listing filed with the application follows.

SEQUENCE LISTING (63 sequences)

SEQ ID NO: 1 - DNA, 6345 bp, Homo sapiens
gtgctgcccgcctagaaagggtgaagtggttgtttccgtgacggactgagtacgggtgcctgtcaggctcttgcggaagtccatgcgccattgggagggcctcggccgcggctctgtgcccttgctgctgagggccacttcctgggtcattcctggaccgggagccgggctggggctcacacgggggctcccgcgtggccgtctcggcgcctgcgtgacctccccgccggcgggatgtggcgactacgtcgggccgctgtggcctgtgaggtctgccagtctttagtgaaacacagctctggaataaaaggaagtttaccactacaaaaactacatctggtttcacgaagcatttatcattcacatcatcctaccttaaagcttcaacgaccccaattaaggacatcctttcagcagttctcttctctgacaaaccttcctttacgtaaactgaaattctctccaattaaatatggctaccagcctcgcaggaatttttggccagcaagattagctacgagactcttaaaacttcgctatctcatactaggatcggctgttgggggtggctacacagccaaaaagacttttgatcagtggaaagatatgataccggaccttagtgaatataaatggattgtgcctgacattgtgtgggaaattgatgagtatatcgattttgagaaaattagaaaagcccttcctagttcagaagaccttgtaaagttagcaccagactttgacaagattgttgaaagccttagcttattgaaggacttttttacctcaggttctccggaagaaacggcgtttagagcaacagatcgtggatctgaaagtgacaagcattttagaaaggtgtcagacaaagagaaaattgaccaacttcaggaagaacttctgcacactcagttgaagtatcagagaatcttggaacgattagaaaaggagaacaaagaattgagaaaattagtattgcagaaagatgacaaaggcattcatcatagaaagcttaagaaatctttgattgacatgtattctgaagttcttgatgttctctctgattatgatgccagttataatacgcaagatcatctgccacgggttgttgtggttggagatcagagtgctggaaagactagtgtgttggaaatgattgcccaagctcgaatattcccaagaggatctggggagatgatgacacgttctccagttaaggtgactctgagtgaaggtcctcaccatgtggccctatttaaagatagttctcgggagtttgatcttaccaaagaagaagatcttgcagcattaagacatgaaatagaacttcgaatgaggaaaaatgtgaaagaaggctgtaccgttagccctgagaccatatccttaaatgtaaaaggccctggactacagaggatggtgcttgttgacttaccaggtgtgattaatactgtgacatcaggcatggctcctgacacaaaggaaactattttcagtatcagcaaagcttacatgcagaatcctaatgccatcatactgtgtattcaagatggatctgtggatgctgaacgcagtattgttacagacttggtcagtcaaatggaccctcatggaaggagaaccatattcgttttgaccaaagtagacctggcagagaaaaatgtagccagtccaagcaggattcagcagataattgaaggaaagctcttcccaatgaaagctttaggttattttgctgttgtaacaggaaaagggaacagctctgaaagcattgaagctataagagaatatgaagaagagttttttcagaattcaaagctcctaaagacaagcatgctaaaggcacaccaagtgactacaagaaatttaagccttgcagtatcagactgcttttggaaaatggtacgagagtctgttgaacaacaggctgatagtttcaaagcaacacgttttaaccttgaaactgaatggaagaataactatcctcgcctgcgggaacttgaccggaatgaactatttgaaaaagctaaaaatgaaatccttgatgaagttatcagtctgagccaggttacaccaaaacattgggaggaaatccttcaacaatctttgtgggaaagagtatcaactcatgtgattgaaaacatctaccttccagctgcgcagaccatgaattcaggaacttttaacaccacagtggatatcaagcttaaacagtggactgataaacaacttcctaataaagcagtagaggttgcttgggagaccctacaagaagaattttcccgctttatgacagaaccgaaagggaaagagcatgatgacatatttgataaacttaaagaggctgttaaggaagaaagtattaaacgacacaagtggaatgactttgcggaggacagcttgagggttattcaacacaatgctttggaagaccgatccatatctgataaacagcaatgggatgcagctatttattttatggaagaggctctgcaggctcgtctcaaggatactgaaaatgcaattgaaaacatggtgggtccagactggaaaaagaggtggttatactggaagaatcggacccaagaacagtgtgttcacaatgaaaccaagaatgaattggagaagatgttgaaatgtaatgaggagcacccagcttatcttgcaagtgatgaaataaccacagtccggaagaaccttgaatcccgaggagtagaagtagatccaagcttgattaaggatacttggcatcaagtttatagaagacattttttaaaaacagctctaaaccattgtaacctttgtcgaagaggtttttattactaccaaaggcattttgtagattctgagttggaatgcaatgatgtggtcttgttttggcgtatacagcgcatgcttgctatcaccgcaaatactttaaggcaacaacttacaaatactgaagttaggcgattagagaaaaatgttaaagaggtattggaagattttgctgaagatggtgagaagaagattaaattgcttactggtaaacgcgttcaactggcggaagacctcaagaaagttagagaaattcaagaaaaacttgatgctttcattgaagctcttcatcaggagaaataaattaaaatcgtactcataatcagctctgcatacatctgaagaacaaaaacatcaacgtcttttgtccagcctctttttcttctgctgttccacctttctaaacatacaataaagtcatgggataaaaataatcgatgtatgttacgggcgctttaaccatcagctgcctctcgaatggaagaacagtggtaatggattaacatcctattttgttgtactaaagtgacaaatcggaataatataattggtatggccattaggttcagtccttgaagataagaaacttgttctctgtttgttgtcttatttgtggtggcactcgtttaatggattaactgaggttgctcaatgttcagtttcttttccagaaatacaatgctaggtgttttgaaataaaacttatatagcaattgtttaaagttatcaattgtatataaaatcacagtagcctgctaaatcattgtatgtgtctgtagtattctattcccagaaactatttgaccatgataattcagtttatattcaccacatgaaagaaaaatgggtaacagaagaacccttaaaacaggttaatttggattgtaacgttcagtgaaagaaatttcaacccttcatagccagcgaagaaatttgccttggaagccaagtcagtaccagcttacctatttgattcagttgctgttttctcactctctatatccatttgaaattgatttattttagatgttgtatacttacgttaggctttctgttaatagtggtttttctcctgttgacagagccaccggattatgacacaggatgaggaagattaaggataatcaattgactaatttcatttagaatattatcaaacatttcaactaggtatcagaaaaaggctttctttcataagactattttaaatagaaattatttcaacaattaaagtaatgttgaccatccccctctcagctgaataaagaaaaatttagttcaatttattgcaatttaattacaatactaccttcacaacattttcatgtgttttaaataaatattttttaattggctaaaggacattcaagcaaagaaatgctttctttacttaaaatgtctatctcatttgctgccttttcactaagcctttactttgttaataaaagtgtccattgtgtgatgtttttgattttacagtttgctaaatcttattttcttggagttgctttttggtaacagccccattgctactccccattttattgttttacatcaatgcatgcttcgttgtgatccctcaagatgtaacacttggtatgctcggttgaggatatgaaaaaatacttccgaaaccaggaattcaatgtatgtttgttttatactgtttgataagaaaagtaggtccagccttaagcagcacagatgcgctggtagatgcatagtcaggaactttttttatttcttttaggtctagggacaggagtgaatagaaagggaggagagctctattatgttctatacacagattaggagatgaccttactgggtacacccctctaaccagtgcttacaggttaatgcatgttaatgaatatttttgcagttgtaaagcataacaattacaactacacatctatttctaaagaataaaacaggaccatatttatttacttctgtcaactatagaaagaaagaccttcagctgtatttccacagatttctcccaaggaaaaggctaatattagtcactactgttatcacatccctttgtataagttttaaaaagagatggagggagatcttcatttctttgaggagatcagtattgtaacgtatgtgaatagatgataacaattaatattactaaaagtcccacatgagagtcctgacgccctctccatgccccacagtaatgtggcttctttcatgggtttttttttcttctttttagctgatctcatcctaagcatgctttatttttccttgaaagctaggtatttatcaactgcagatgttattgaaagaaaataaaattcagtctcaagagtaaaccctgtgtcttgtgtctgtagttcaaaagtcagaaatgattctaatttaaacaaaaagatactaaatatacagaagttaaattcgaactagccacagaatcatttgtttttatgtcagaatttgcaaagagtggagtggacaaagctctgtatggaagactgaacaactgtaaatagatgatatccaaacttaatttggctaggacttcaattttaaaaatcagtgtacctaggcagtgcacagcacgaaataagtggcccttgcagcttccccgtttaacccactgtgctatagttgcgggtggaacagtcaacctttctagtagtttatgatattgccctctttgtattcccattttctacagttttttccgcagacttctttctgcaaattattcagcctccaaatgcaaatgaatgatataaaaataagtagggaacatggcagagagtggtgcttcccagcctcacaatgtgggaatttgacataggatgagagtcagagtataggtttaaaagataaaatctttagttaataattttgtatttatttattctagatgtatgtatctgaggaaagaaatctggtatttttgctttccaataaaggggatcaaagtaatggtttttctctcagttctctaagctggtctatgttatagctctagcagtatggaaatgtgctttaaaatatgcttaccttttgaatgatcatggctatatgttgttgagatatttgaaacttaccttgttttcacttgtgcactgtgaatgaactttgtattatttttttaaaaccttcacattacgtgtagatattattgcaacttatattttgcctgagcttgatcaaaggtcatttgtgtagatgagtaattaaaaaatatttaaatcacattataattctattattggagagcatcttttaaatttttttctgttttaacgagggaaagagaaacctgtatacctagggtcattatttgaccccatagtataaccagattcatggtctaacaagctctcagtgtggcttttctctgaatgcttgaatttcacatgccttgcatttcacagttgtactccatggtcaaccggtgctttttttcacatcgtggtacttgtcaaaacattttgttattttccttggtaaaatatataaaaaaggttttctaatttcaaaaaaaaaaaaaaaaaa

SEQ ID NO: 2 - protein, 960 aa, Homo sapiens
MWRLRRAAVACEVCQSLVKHSSGIKGSLPLQKLHLVSRSIYHSHHPTLKLQRPQLRTSFQQFSSLTNLPLRKLKFSPIKYGYQPRRNFWPARLATRLLKLRYLILGSAVGGGYTAKKTFDQWKDMIPDLSEYKWIVPDIVWEIDEYIDFEKIRKALPSSEDLVKLAPDFDKIVESLSLLKDFFTSGSPEETAFRATDRGSESDKHFRKVSDKEKIDQLQEELLHTQLKYQRILERLEKENKELRKLVLQKDDKGIHHRKLKKSLIDMYSEVLDVLSDYDASYNTQDHLPRVVVVGDQSAGKTSVLEMIAQARIFPRGSGEMMTRSPVKVTLSEGPHHVALFKDSSREFDLTKEEDLAALRHEIELRMRKNVKEGCTVSPETISLNVKGPGLQRMVLVDLPGVINTVTSGMAPDTKETIFSISKAYMQNPNAIILCIQDGSVDAERSIVTDLVSQMDPHGRRTIFVLTKVDLAEKNVASPSRIQQIIEGKLFPMKALGYFAVVTGKGNSSESIEAIREYEEEFFQNSKLLKTSMLKAHQVTTRNLSLAVSDCFWKMVRESVEQQADSFKATRFNLETEWKNNYPRLRELDRNELFEKAKNEILDEVISLSQVTPKHWEEILQQSLWERVSTHVIENIYLPAAQTMNSGTFNTTVDIKLKQWTDKQLPNKAVEVAWETLQEEFSRFMTEPKGKEHDDIFDKLKEAVKEESIKRHKWNDFAEDSLRVIQHNALEDRSISDKQQWDAAIYFMEEALQARLKDTENAIENMVGPDWKKRWLYWKNRTQEQCVHNETKNELEKMLKCNEEHPAYLASDEITTVRKNLESRGVEVDPSLIKDTWHQVYRRHFLKTALNHCNLCRRGFYYYQRHFVDSELECNDVVLFWRIQRMLAITANTLRQQLTNTEVRRLEKNVKEVLEDFAEDGEKKIKLLTGKRVQLAEDLKKVREIQEKLDAFIEALHQEK

SEQ ID NO: 3 - DNA, 6237 bp, Homo sapiens
gtgctgcccgcctagaaagggtgaagtggttgtttccgtgacggactgagtacgggtgcctgtcaggctcttgcggaagtccatgcgccattgggagggcctcggccgcggctctgtgcccttgctgctgagggccacttcctgggtcattcctggaccgggagccgggctggggctcacacgggggctcccgcgtggccgtctcggcgcctgcgtgacctccccgccggcgggatgtggcgactacgtcgggccgctgtggcctgtgaggtctgccagtctttagtgaaacacagctctggaataaaaggaagtttaccactacaaaaactacatctggtttcacgaagcatttatcattcacatcatcctaccttaaagcttcaacgaccccaattaaggacatcctttcagcagttctcttctctgacaaaccttcctttacgtaaactgaaattctctccaattaaatatggctaccagcctcgcaggaatttttggccagcaagattagctacgagactcttaaaacttcgctatctcatactaggatcggctgttgggggtggctacacagccaaaaagacttttgatcagtggaaagatatgataccggaccttagtgaatataaatggattgtgcctgacattgtgtgggaaattgatgagtatatcgattttggttctccggaagaaacggcgtttagagcaacagatcgtggatctgaaagtgacaagcattttagaaaggtgtcagacaaagagaaaattgaccaacttcaggaagaacttctgcacactcagttgaagtatcagagaatcttggaacgattagaaaaggagaacaaagaattgagaaaattagtattgcagaaagatgacaaaggcattcatcatagaaagcttaagaaatctttgattgacatgtattctgaagttcttgatgttctctctgattatgatgccagttataatacgcaagatcatctgccacgggttgttgtggttggagatcagagtgctggaaagactagtgtgttggaaatgattgcccaagctcgaatattcccaagaggatctggggagatgatgacacgttctccagttaaggtgactctgagtgaaggtcctcaccatgtggccctatttaaagatagttctcgggagtttgatcttaccaaagaagaagatcttgcagcattaagacatgaaatagaacttcgaatgaggaaaaatgtgaaagaaggctgtaccgttagccctgagaccatatccttaaatgtaaaaggccctggactacagaggatggtgcttgttgacttaccaggtgtgattaatactgtgacatcaggcatggctcctgacacaaaggaaactattttcagtatcagcaaagcttacatgcagaatcctaatgccatcatactgtgtattcaagatggatctgtggatgctgaacgcagtattgttacagacttggtcagtcaaatggaccctcatggaaggagaaccatattcgttttgaccaaagtagacctggcagagaaaaatgtagccagtccaagcaggattcagcagataattgaaggaaagctcttcccaatgaaagctttaggttattttgctgttgtaacaggaaaagggaacagctctgaaagcattgaagctataagagaatatgaagaagagttttttcagaattcaaagctcctaaagacaagcatgctaaaggcacaccaagtgactacaagaaatttaagccttgcagtatcagactgcttttggaaaatggtacgagagtctgttgaacaacaggctgatagtttcaaagcaacacgttttaaccttgaaactgaatggaagaataactatcctcgcctgcgggaacttgaccggaatgaactatttgaaaaagctaaaaatgaaatccttgatgaagttatcagtctgagccaggttacaccaaaacattgggaggaaatccttcaacaatctttgtgggaaagagtatcaactcatgtgattgaaaacatctaccttccagctgcgcagaccatgaattcaggaacttttaacaccacagtggatatcaagcttaaacagtggactgataaacaacttcctaataaagcagtagaggttgcttgggagaccctacaagaagaattttcccgctttatgacagaaccgaaagggaaagagcatgatgacatatttgataaacttaaagaggctgttaaggaagaaagtattaaacgacacaagtggaatgactttgcggaggacagcttgagggttattcaacacaatgctttggaagaccgatccatatctgataaacagcaatgggatgcagctatttattttatggaagaggctctgcaggctcgtctcaaggatactgaaaatgcaattgaaaacatggtgggtccagactggaaaaagaggtggttatactggaagaatcggacccaagaacagtgtgttcacaatgaaaccaagaatgaattggagaagatgttgaaatgtaatgaggagcacccagcttatcttgcaagtgatgaaataaccacagtccggaagaaccttgaatcccgaggagtagaagtagatccaagcttgattaaggatacttggcatcaagtttatagaagacattttttaaaaacagctctaaaccattgtaacctttgtcgaagaggtttttattactaccaaaggcattttgtagattctgagttggaatgcaatgatgtggtcttgttttggcgtatacagcgcatgcttgctatcaccgcaaatactttaaggcaacaacttacaaatactgaagttaggcgattagagaaaaatgttaaagaggtattggaagattttgctgaagatggtgagaagaagattaaattgcttactggtaaacgcgttcaactggcggaagacctcaagaaagttagagaaattcaagaaaaacttgatgctttcattgaagctcttcatcaggagaaataaattaaaatcgtactcataatcagctctgcatacatctgaagaacaaaaacatcaacgtcttttgtccagcctctttttcttctgctgttccacctttctaaacatacaataaagtcatgggataaaaataatcgatgtatgttacgggcgctttaaccatcagctgcctctcgaatggaagaacagtggtaatggattaacatcctattttgttgtactaaagtgacaaatcggaataatataattggtatggccattaggttcagtccttgaagataagaaacttgttctctgtttgttgtcttatttgtggtggcactcgtttaatggattaactgaggttgctcaatgttcagtttcttttccagaaatacaatgctaggtgttttgaaataaaacttatatagcaattgtttaaagttatcaattgtatataaaatcacagtagcctgctaaatcattgtatgtgtctgtagtattctattcccagaaactatttgaccatgataattcagtttatattcaccacatgaaagaaaaatgggtaacagaagaacccttaaaacaggttaatttggattgtaacgttcagtgaaagaaatttcaacccttcatagccagcgaagaaatttgccttggaagccaagtcagtaccagcttacctatttgattcagttgctgttttctcactctctatatccatttgaaattgatttattttagatgttgtatacttacgttaggctttctgttaatagtggtttttctcctgttgacagagccaccggattatgacacaggatgaggaagattaaggataatcaattgactaatttcatttagaatattatcaaacatttcaactaggtatcagaaaaaggctttctttcataagactattttaaatagaaattatttcaacaattaaagtaatgttgaccatccccctctcagctgaataaagaaaaatttagttcaatttattgcaatttaattacaatactaccttcacaacattttcatgtgttttaaataaatattttttaattggctaaaggacattcaagcaaagaaatgctttctttacttaaaatgtctatctcatttgctgccttttcactaagcctttactttgttaataaaagtgtccattgtgtgatgtttttgattttacagtttgctaaatcttattttcttggagttgctttttggtaacagccccattgctactccccattttattgttttacatcaatgcatgcttcgttgtgatccctcaagatgtaacacttggtatgctcggttgaggatatgaaaaaatacttccgaaaccaggaattcaatgtatgtttgttttatactgtttgataagaaaagtaggtccagccttaagcagcacagatgcgctggtagatgcatagtcaggaactttttttatttcttttaggtctagggacaggagtgaatagaaagggaggagagctctattatgttctatacacagattaggagatgaccttactgggtacacccctctaaccagtgcttacaggttaatgcatgttaatgaatatttttgcagttgtaaagcataacaattacaactacacatctatttctaaagaataaaacaggaccatatttatttacttctgtcaactatagaaagaaagaccttcagctgtatttccacagatttctcccaaggaaaaggctaatattagtcactactgttatcacatccctttgtataagttttaaaaagagatggagggagatcttcatttctttgaggagatcagtattgtaacgtatgtgaatagatgataacaattaatattactaaaagtcccacatgagagtcctgacgccctctccatgccccacagtaatgtggcttctttcatgggtttttttttcttctttttagctgatctcatcctaagcatgctttatttttccttgaaagctaggtatttatcaactgcagatgttattgaaagaaaataaaattcagtctcaagagtaaaccctgtgtcttgtgtctgtagttcaaaagtcagaaatgattctaatttaaacaaaaagatactaaatatacagaagttaaattcgaactagccacagaatcatttgtttttatgtcagaatttgcaaagagtggagtggacaaagctctgtatggaagactgaacaactgtaaatagatgatatccaaacttaatttggctaggacttcaattttaaaaatcagtgtacctaggcagtgcacagcacgaaataagtggcccttgcagcttccccgtttaacccactgtgctatagttgcgggtggaacagtcaacctttctagtagtttatgatattgccctctttgtattcccattttctacagttttttccgcagacttctttctgcaaattattcagcctccaaatgcaaatgaatgatataaaaataagtagggaacatggcagagagtggtgcttcccagcctcacaatgtgggaatttgacataggatgagagtcagagtataggtttaaaagataaaatctttagttaataattttgtatttatttattctagatgtatgtatctgaggaaagaaatctggtatttttgctttccaataaaggggatcaaagtaatggtttttctctcagttctctaagctggtctatgttatagctctagcagtatggaaatgtgctttaaaatatgcttaccttttgaatgatcatggctatatgttgttgagatatttgaaacttaccttgttttcacttgtgcactgtgaatgaactttgtattatttttttaaaaccttcacattacgtgtagatattattgcaacttatattttgcctgagcttgatcaaaggtcatttgtgtagatgagtaattaaaaaatatttaaatcacattataattctattattggagagcatcttttaaatttttttctgttttaacgagggaaagagaaacctgtatacctagggtcattatttgaccccatagtataaccagattcatggtctaacaagctctcagtgtggcttttctctgaatgcttgaatttcacatgccttgcatttcacagttgtactccatggtcaaccggtgctttttttcacatcgtggtacttgtcaaaacattttgttattttccttggtaaaatatataaaaaaggttttctaatttcaaaaaaaaaaaaaaaaaa

SEQ ID NO: 4 - protein, 924 aa, Homo sapiens
MWRLRRAAVACEVCQSLVKHSSGIKGSLPLQKLHLVSRSIYHSHHPTLKLQRPQLRTSFQQFSSLTNLPLRKLKFSPIKYGYQPRRNFWPARLATRLLKLRYLILGSAVGGGYTAKKTFDQWKDMIPDLSEYKWIVPDIVWEIDEYIDFGSPEETAFRATDRGSESDKHFRKVSDKEKIDQLQEELLHTQLKYQRILERLEKENKELRKLVLQKDDKGIHHRKLKKSLIDMYSEVLDVLSDYDASYNTQDHLPRVVVVGDQSAGKTSVLEMIAQARIFPRGSGEMMTRSPVKVTLSEGPHHVALFKDSSREFDLTKEEDLAALRHEIELRMRKNVKEGCTVSPETISLNVKGPGLQRMVLVDLPGVINTVTSGMAPDTKETIFSISKAYMQNPNAIILCIQDGSVDAERSIVTDLVSQMDPHGRRTIFVLTKVDLAEKNVASPSRIQQIIEGKLFPMKALGYFAVVTGKGNSSESIEAIREYEEEFFQNSKLLKTSMLKAHQVTTRNLSLAVSDCFWKMVRESVEQQADSFKATRFNLETEWKNNYPRLRELDRNELFEKAKNEILDEVISLSQVTPKHWEEILQQSLWERVSTHVIENIYLPAAQTMNSGTFNTTVDIKLKQWTDKQLPNKAVEVAWETLQEEFSRFMTEPKGKEHDDIFDKLKEAVKEESIKRHKWNDFAEDSLRVIQHNALEDRSISDKQQWDAAIYFMEEALQARLKDTENAIENMVGPDWKKRWLYWKNRTQEQCVHNETKNELEKMLKCNEEHPAYLASDEITTVRKNLESRGVEVDPSLIKDTWHQVYRRHFLKTALNHCNLCRRGFYYYQRHFVDSELECNDVVLFWRIQRMLAITANTLRQQLTNTEVRRLEKNVKEVLEDFAEDGEKKIKLLTGKRVQLAEDLKKVREIQEKLDAFIEALHQEK

SEQ ID NO: 5 - DNA, 6291 bp, Homo sapiens
gtgctgcccgcctagaaagggtgaagtggttgtttccgtgacggactgagtacgggtgcctgtcaggctcttgcggaagtccatgcgccattgggagggcctcggccgcggctctgtgcccttgctgctgagggccacttcctgggtcattcctggaccgggagccgggctggggctcacacgggggctcccgcgtggccgtctcggcgcctgcgtgacctccccgccggcgggatgtggcgactacgtcgggccgctgtggcctgtgaggtctgccagtctttagtgaaacacagctctggaataaaaggaagtttaccactacaaaaactacatctggtttcacgaagcatttatcattcacatcatcctaccttaaagcttcaacgaccccaattaaggacatcctttcagcagttctcttctctgacaaaccttcctttacgtaaactgaaattctctccaattaaatatggctaccagcctcgcaggaatttttggccagcaagattagctacgagactcttaaaacttcgctatctcatactaggatcggctgttgggggtggctacacagccaaaaagacttttgatcagtggaaagatatgataccggaccttagtgaatataaatggattgtgcctgacattgtgtgggaaattgatgagtatatcgattttggtcacaaattggttagtgaagtcataggagcttctgacctacttctcttgttaggttctccggaagaaacggcgtttagagcaacagatcgtggatctgaaagtgacaagcattttagaaaggtgtcagacaaagagaaaattgaccaacttcaggaagaacttctgcacactcagttgaagtatcagagaatcttggaacgattagaaaaggagaacaaagaattgagaaaattagtattgcagaaagatgacaaaggcattcatcatagaaagcttaagaaatctttgattgacatgtattctgaagttcttgatgttctctctgattatgatgccagttataatacgcaagatcatctgccacgggttgttgtggttggagatcagagtgctggaaagactagtgtgttggaaatgattgcccaagctcgaatattcccaagaggatctggggagatgatgacacgttctccagttaaggtgactctgagtgaaggtcctcaccatgtggccctatttaaagatagttctcgggagtttgatcttaccaaagaagaagatcttgcagcattaagacatgaaatagaacttcgaatgaggaaaaatgtgaaagaaggctgtaccgttagccctgagaccatatccttaaatgtaaaaggccctggactacagaggatggtgcttgttgacttaccaggtgtgattaatactgtgacatcaggcatggctcctgacacaaaggaaactattttcagtatcagcaaagcttacatgcagaatcctaatgccatcatactgtgtattcaagatggatctgtggatgctgaacgcagtattgttacagacttggtcagtcaaatggaccctcatggaaggagaaccatattcgttttgaccaaagtagacctggcagagaaaaatgtagccagtccaagcaggattcagcagataattgaaggaaagctcttcccaatgaaagctttaggttattttgctgttgtaacaggaaaagggaacagctctgaaagcattgaagctataagagaatatgaagaagagttttttcagaattcaaagctcctaaagacaagcatgctaaaggcacaccaagtgactacaagaaatttaagccttgcagtatcagactgcttttggaaaatggtacgagagtctgttgaacaacaggctgatagtttcaaagcaacacgttttaaccttgaaactgaatggaagaataactatcctcgcctgcgggaacttgaccggaatgaactatttgaaaaagctaaaaatgaaatccttgatgaagttatcagtctgagccaggttacaccaaaacattgggaggaaatccttcaacaatctttgtgggaaagagtatcaactcatgtgattgaaaacatctaccttccagctgcgcagaccatgaattcaggaacttttaacaccacagtggatatcaagcttaaacagtggactgataaacaacttcctaataaagcagtagaggttgcttgggagaccctacaagaagaattttcccgctttatgacagaaccgaaagggaaagagcatgatgacatatttgataaacttaaagaggctgttaaggaagaaagtattaaacgacacaagtggaatgactttgcggaggacagcttgagggttattcaacacaatgctttggaagaccgatccatatctgataaacagcaatgggatgcagctatttattttatggaagaggctctgcaggctcgtctcaaggatactgaaaatgcaattgaaaacatggtgggtccagactggaaaaagaggtggttatactggaagaatcggacccaagaacagtgtgttcacaatgaaaccaagaatgaattggagaagatgttgaaatgtaatgaggagcacccagcttatcttgcaagtgatgaaataaccacagtccggaagaaccttgaatcccgaggagtagaagtagatccaagcttgattaaggatacttggcatcaagtttatagaagacattttttaaaaacagctctaaaccattgtaacctttgtcgaagaggtttttattactaccaaaggcattttgtagattctgagttggaatgcaatgatgtggtcttgttttggcgtatacagcgcatgcttgctatcaccgcaaatactttaaggcaacaacttacaaatactgaagttaggcgattagagaaaaatgttaaagaggtattggaagattttgctgaagatggtgagaagaagattaaattgcttactggtaaacgcgttcaactggcggaagacctcaagaaagttagagaaattcaagaaaaacttgatgctttcattgaagctcttcatcaggagaaataaattaaaatcgtactcataatcagctctgcatacatctgaagaacaaaaacatcaacgtcttttgtccagcctctttttcttctgctgttccacctttctaaacatacaataaagtcatgggataaaaataatcgatgtatgttacgggcgctttaaccatcagctgcctctcgaatggaagaacagtggtaatggattaacatcctattttgttgtactaaagtgacaaatcggaataatataattggtatggccattaggttcagtccttgaagataagaaacttgttctctgtttgttgtcttatttgtggtggcactcgtttaatggattaactgaggttgctcaatgttcagtttcttttccagaaatacaatgctaggtgttttgaaataaaacttatatagcaattgtttaaagttatcaattgtatataaaatcacagtagcctgctaaatcattgtatgtgtctgtagtattctattcccagaaactatttgaccatgataattcagtttatattcaccacatgaaagaaaaatgggtaacagaagaacccttaaaacaggttaatttggattgtaacgttcagtgaaagaaatttcaacccttcatagccagcgaagaaatttgccttggaagccaagtcagtaccagcttacctatttgattcagttgctgttttctcactctctatatccatttgaaattgatttattttagatgttgtatacttacgttaggctttctgttaatagtggtttttctcctgttgacagagccaccggattatgacacaggatgaggaagattaaggataatcaattgactaatttcatttagaatattatcaaacatttcaactaggtatcagaaaaaggctttctttcataagactattttaaatagaaattatttcaacaattaaagtaatgttgaccatccccctctcagctgaataaagaaaaatttagttcaatttattgcaatttaattacaatactaccttcacaacattttcatgtgttttaaataaatattttttaattggctaaaggacattcaagcaaagaaatgctttctttacttaaaatgtctatctcatttgctgccttttcactaagcctttactttgttaataaaagtgtccattgtgtgatgtttttgattttacagtttgctaaatcttattttcttggagttgctttttggtaacagccccattgctactccccattttattgttttacatcaatgcatgcttcgttgtgatccctcaagatgtaacacttggtatgctcggttgaggatatgaaaaaatacttccgaaaccaggaattcaatgtatgtttgttttatactgtttgataagaaaagtaggtccagccttaagcagcacagatgcgctggtagatgcatagtcaggaactttttttatttcttttaggtctagggacaggagtgaatagaaagggaggagagctctattatgttctatacacagattaggagatgaccttactgggtacacccctctaaccagtgcttacaggttaatgcatgttaatgaatatttttgcagttgtaaagcataacaattacaactacacatctatttctaaagaataaaacaggaccatatttatttacttctgtcaactatagaaagaaagaccttcagctgtatttccacagatttctcccaaggaaaaggctaatattagtcactactgttatcacatccctttgtataagttttaaaaagagatggagggagatcttcatttctttgaggagatcagtattgtaacgtatgtgaatagatgataacaattaatattactaaaagtcccacatgagagtcctgacgccctctccatgccccacagtaatgtggcttctttcatgggtttttttttcttctttttagctgatctcatcctaagcatgctttatttttccttgaaagctaggtatttatcaactgcagatgttattgaaagaaaataaaattcagtctcaagagtaaaccctgtgtcttgtgtctgtagttcaaaagtcagaaatgattctaatttaaacaaaaagatactaaatatacagaagttaaattcgaactagccacagaatcatttgtttttatgtcagaatttgcaaagagtggagtggacaaagctctgtatggaagactgaacaactgtaaatagatgatatccaaacttaatttggctaggacttcaattttaaaaatcagtgtacctaggcagtgcacagcacgaaataagtggcccttgcagcttccccgtttaacccactgtgctatagttgcgggtggaacagtcaacctttctagtagtttatgatattgccctctttgtattcccattttctacagttttttccgcagacttctttctgcaaattattcagcctccaaatgcaaatgaatgatataaaaataagtagggaacatggcagagagtggtgcttcccagcctcacaatgtgggaatttgacataggatgagagtcagagtataggtttaaaagataaaatctttagttaataattttgtatttatttattctagatgtatgtatctgaggaaagaaatctggtatttttgctttccaataaaggggatcaaagtaatggtttttctctcagttctctaagctggtctatgttatagctctagcagtatggaaatgtgctttaaaatatgcttaccttttgaatgatcatggctatatgttgttgagatatttgaaacttaccttgttttcacttgtgcactgtgaatgaactttgtattatttttttaaaaccttcacattacgtgtagatattattgcaacttatattttgcctgagcttgatcaaaggtcatttgtgtagatgagtaattaaaaaatatttaaatcacattataattctattattggagagcatcttttaaatttttttctgttttaacgagggaaagagaaacctgtatacctagggtcattatttgaccccatagtataaccagattcatggtctaacaagctctcagtgtggcttttctctgaatgcttgaatttcacatgccttgcatttcacagttgtactccatggtcaaccggtgctttttttcacatcgtggtacttgtcaaaacattttgttattttccttggtaaaatatataaaaaaggttttctaatttcaaaaaaaaaaaaaaaaaa

SEQ ID NO: 6 - protein, 942 aa, Homo sapiens
MWRLRRAAVACEVCQSLVKHSSGIKGSLPLQKLHLVSRSIYHSHHPTLKLQRPQLRTSFQQFSSLTNLPLRKLKFSPIKYGYQPRRNFWPARLATRLLKLRYLILGSAVGGGYTAKKTFDQWKDMIPDLSEYKWIVPDIVWEIDEYIDFGHKLVSEVIGASDLLLLLGSPEETAFRATDRGSESDKHFRKVSDKEKIDQLQEELLHTQLKYQRILERLEKENKELRKLVLQKDDKGIHHRKLKKSLIDMYSEVLDVLSDYDASYNTQDHLPRVVVVGDQSAGKTSVLEMIAQARIFPRGSGEMMTRSPVKVTLSEGPHHVALFKDSSREFDLTKEEDLAALRHEIELRMRKNVKEGCTVSPETISLNVKGPGLQRMVLVDLPGVINTVTSGMAPDTKETIFSISKAYMQNPNAIILCIQDGSVDAERSIVTDLVSQMDPHGRRTIFVLTKVDLAEKNVASPSRIQQIIEGKLFPMKALGYFAVVTGKGNSSESIEAIREYEEEFFQNSKLLKTSMLKAHQVTTRNLSLAVSDCFWKMVRESVEQQADSFKATRFNLETEWKNNYPRLRELDRNELFEKAKNEILDEVISLSQVTPKHWEEILQQSLWERVSTHVIENIYLPAAQTMNSGTFNTTVDIKLKQWTDKQLPNKAVEVAWETLQEEFSRFMTEPKGKEHDDIFDKLKEAVKEESIKRHKWNDFAEDSLRVIQHNALEDRSISDKQQWDAAIYFMEEALQARLKDTENAIENMVGPDWKKRWLYWKNRTQEQCVHNETKNELEKMLKCNEEHPAYLASDEITTVRKNLESRGVEVDPSLIKDTWHQVYRRHFLKTALNHCNLCRRGFYYYQRHFVDSELECNDVVLFWRIQRMLAITANTLRQQLTNTEVRRLEKNVKEVLEDFAEDGEKKIKLLTGKRVQLAEDLKKVREIQEKLDAFIEALHQEK

SEQ ID NO: 7 - DNA, 6348 bp, Homo sapiens
gtgctgcccgcctagaaagggtgaagtggttgtttccgtgacggactgagtacgggtgcctgtcaggctcttgcggaagtccatgcgccattgggagggcctcggccgcggctctgtgcccttgctgctgagggccacttcctgggtcattcctggaccgggagccgggctggggctcacacgggggctcccgcgtggccgtctcggcgcctgcgtgacctccccgccggcgggatgtggcgactacgtcgggccgctgtggcctgtgaggtctgccagtctttagtgaaacacagctctggaataaaaggaagtttaccactacaaaaactacatctggtttcacgaagcatttatcattcacatcatcctaccttaaagcttcaacgaccccaattaaggacatcctttcagcagttctcttctctgacaaaccttcctttacgtaaactgaaattctctccaattaaatatggctaccagcctcgcaggaatttttggccagcaagattagctacgagactcttaaaacttcgctatctcatactaggatcggctgttgggggtggctacacagccaaaaagacttttgatcagtggaaagatatgataccggaccttagtgaatataaatggattgtgcctgacattgtgtgggaaattgatgagtatatcgattttggttctccggaagaaacggcgtttagagcaacagatcgtggatctgaaagtgacaagcattttagaaagggtctgcttggtgagctcattctcttacaacaacaaattcaagagcatgaagaggaagcgcgcagagccgctggccaatatagcacgagctatgcccaacagaagcgcaaggtgtcagacaaagagaaaattgaccaacttcaggaagaacttctgcacactcagttgaagtatcagagaatcttggaacgattagaaaaggagaacaaagaattgagaaaattagtattgcagaaagatgacaaaggcattcatcatagaaagcttaagaaatctttgattgacatgtattctgaagttcttgatgttctctctgattatgatgccagttataatacgcaagatcatctgccacgggttgttgtggttggagatcagagtgctggaaagactagtgtgttggaaatgattgcccaagctcgaatattcccaagaggatctggggagatgatgacacgttctccagttaaggtgactctgagtgaaggtcctcaccatgtggccctatttaaagatagttctcgggagtttgatcttaccaaagaagaagatcttgcagcattaagacatgaaatagaacttcgaatgaggaaaaatgtgaaagaaggctgtaccgttagccctgagaccatatccttaaatgtaaaaggccctggactacagaggatggtgcttgttgacttaccaggtgtgattaatactgtgacatcaggcatggctcctgacacaaaggaaactattttcagtatcagcaaagcttacatgcagaatcctaatgccatcatactgtgtattcaagatggatctgtggatgctgaacgcagtattgttacagacttggtcagtcaaatggaccctcatggaaggagaaccatattcgttttgaccaaagtagacctggcagagaaaaatgtagccagtccaagcaggattcagcagataattgaaggaaagctcttcccaatgaaagctttaggttattttgctgttgtaacaggaaaagggaacagctctgaaagcattgaagctataagagaatatgaagaagagttttttcagaattcaaagctcctaaagacaagcatgctaaaggcacaccaagtgactacaagaaatttaagccttgcagtatcagactgcttttggaaaatggtacgagagtctgttgaacaacaggctgatagtttcaaagcaacacgttttaaccttgaaactgaatggaagaataactatcctcgcctgcgggaacttgaccggaatgaactatttgaaaaagctaaaaatgaaatccttgatgaagttatcagtctgagccaggttacaccaaaacattgggaggaaatccttcaacaatctttgtgggaaagagtatcaactcatgtgattgaaaacatctaccttccagctgcgcagaccatgaattcaggaacttttaacaccacagtggatatcaagcttaaacagtggactgataaacaacttcctaataaagcagtagaggttgcttgggagaccctacaagaagaattttcccgctttatgacagaaccgaaagggaaagagcatgatgacatatttgataaacttaaagaggctgttaaggaagaaagtattaaacgacacaagtggaatgactttgcggaggacagcttgagggttattcaacacaatgctttggaagaccgatccatatctgataaacagcaatgggatgcagctatttattttatggaagaggctctgcaggctcgtctcaaggatactgaaaatgcaattgaaaacatggtgggtccagactggaaaaagaggtggttatactggaagaatcggacccaagaacagtgtgttcacaatgaaaccaagaatgaattggagaagatgttgaaatgtaatgaggagcacccagcttatcttgcaagtgatgaaataaccacagtccggaagaaccttgaatcccgaggagtagaagtagatccaagcttgattaaggatacttggcatcaagtttatagaagacattttttaaaaacagctctaaaccattgtaacctttgtcgaagaggtttttattactaccaaaggcattttgtagattctgagttggaatgcaatgatgtggtcttgttttggcgtatacagcgcatgcttgctatcaccgcaaatactttaaggcaacaacttacaaatactgaagttaggcgattagagaaaaatgttaaagaggtattggaagattttgctgaagatggtgagaagaagattaaattgcttactggtaaacgcgttcaactggcggaagacctcaagaaagttagagaaattcaagaaaaacttgatgctttcattgaagctcttcatcaggagaaataaattaaaatcgtactcataatcagctctgcatacatctgaagaacaaaaacatcaacgtcttttgtccagcctctttttcttctgctgttccacctttctaaacatacaataaagtcatgggataaaaataatcgatgtatgttacgggcgctttaaccatcagctgcctctcgaatggaagaacagtggtaatggattaacatcctattttgttgtactaaagtgacaaatcggaataatataattggtatggccattaggttcagtccttgaagataagaaacttgttctctgtttgttgtcttatttgtggtggcactcgtttaatggattaactgaggttgctcaatgttcagtttcttttccagaaatacaatgctaggtgttttgaaataaaacttatatagcaattgtttaaagttatcaattgtatataaaatcacagtagcctgctaaatcattgtatgtgtctgtagtattctattcccagaaactatttgaccatgataattcagtttatattcaccacatgaaagaaaaatgggtaacagaagaacccttaaaacaggttaatttggattgtaacgttcagtgaaagaaatttcaacccttcatagccagcgaagaaatttgccttggaagccaagtcagtaccagcttacctatttgattcagttgctgttttctcactctctatatccatttgaaattgatttattttagatgttgtatacttacgttaggctttctgttaatagtggtttttctcctgttgacagagccaccggattatgacacaggatgaggaagattaaggataatcaattgactaatttcatttagaatattatcaaacatttcaactaggtatcagaaaaaggctttctttcataagactattttaaatagaaattatttcaacaattaaagtaatgttgaccatccccctctcagctgaataaagaaaaatttagttcaatttattgcaatttaattacaatactaccttcacaacattttcatgtgttttaaataaatattttttaattggctaaaggacattcaagcaaagaaatgctttctttacttaaaatgtctatctcatttgctgccttttcactaagcctttactttgttaataaaagtgtccattgtgtgatgtttttgattttacagtttgctaaatcttattttcttggagttgctttttggtaacagccccattgctactccccattttattgttttacatcaatgcatgcttcgttgtgatccctcaagatgtaacacttggtatgctcggttgaggatatgaaaaaatacttccgaaaccaggaattcaatgtatgtttgttttatactgtttgataagaaaagtaggtccagccttaagcagcacagatgcgctggtagatgcatagtcaggaactttttttatttcttttaggtctagggacaggagtgaatagaaagggaggagagctctattatgttctatacacagattaggagatgaccttactgggtacacccctctaaccagtgcttacaggttaatgcatgttaatgaatatttttgcagttgtaaagcataacaattacaactacacatctatttctaaagaataaaacaggaccatatttatttacttctgtcaactatagaaagaaagaccttcagctgtatttccacagatttctcccaaggaaaaggctaatattagtcactactgttatcacatccctttgtataagttttaaaaagagatggagggagatcttcatttctttgaggagatcagtattgtaacgtatgtgaatagatgataacaattaatattactaaaagtcccacatgagagtcctgacgccctctccatgccccacagtaatgtggcttctttcatgggtttttttttcttctttttagctgatctcatcctaagcatgctttatttttccttgaaagctaggtatttatcaactgcagatgttattgaaagaaaataaaattcagtctcaagagtaaaccctgtgtcttgtgtctgtagttcaaaagtcagaaatgattctaatttaaacaaaaagatactaaatatacagaagttaaattcgaactagccacagaatcatttgtttttatgtcagaatttgcaaagagtggagtggacaaagctctgtatggaagactgaacaactgtaaatagatgatatccaaacttaatttggctaggacttcaattttaaaaatcagtgtacctaggcagtgcacagcacgaaataagtggcccttgcagcttccccgtttaacccactgtgctatagttgcgggtggaacagtcaacctttctagtagtttatgatattgccctctttgtattcccattttctacagttttttccgcagacttctttctgcaaattattcagcctccaaatgcaaatgaatgatataaaaataagtagggaacatggcagagagtggtgcttcccagcctcacaatgtgggaatttgacataggatgagagtcagagtataggtttaaaagataaaatctttagttaataattttgtatttatttattctagatgtatgtatctgaggaaagaaatctggtatttttgctttccaataaaggggatcaaagtaatggtttttctctcagttctctaagctggtctatgttatagctctagcagtatggaaatgtgctttaaaatatgcttaccttttgaatgatcatggctatatgttgttgagatatttgaaacttaccttgttttcacttgtgcactgtgaatgaactttgtattatttttttaaaaccttcacattacgtgtagatattattgcaacttatattttgcctgagcttgatcaaaggtcatttgtgtagatgagtaattaaaaaatatttaaatcacattataattctattattggagagcatcttttaaatttttttctgttttaacgagggaaagagaaacctgtatacctagggtcattatttgaccccatagtataaccagattcatggtctaacaagctctcagtgtggcttttctctgaatgcttgaatttcacatgccttgcatttcacagttgtactccatggtcaaccggtgctttttttcacatcgtggtacttgtcaaaacattttgttattttccttggtaaaatatataaaaaaggttttctaatttcaaaaaaaaaaaaaaaaaa

SEQ ID NO: 8 - protein, 961 aa, Homo sapiens
MWRLRRAAVACEVCQSLVKHSSGIKGSLPLQKLHLVSRSIYHSHHPTLKLQRPQLRTSFQQFSSLTNLPLRKLKFSPIKYGYQPRRNFWPARLATRLLKLRYLILGSAVGGGYTAKKTFDQWKDMIPDLSEYKWIVPDIVWEIDEYIDFGSPEETAFRATDRGSESDKHFRKGLLGELILLQQQIQEHEEEARRAAGQYSTSYAQQKRKVSDKEKIDQLQEELLHTQLKYQRILERLEKENKELRKLVLQKDDKGIHHRKLKKSLIDMYSEVLDVLSDYDASYNTQDHLPRVVVVGDQSAGKTSVLEMIAQARIFPRGSGEMMTRSPVKVTLSEGPHHVALFKDSSREFDLTKEEDLAALRHEIELRMRKNVKEGCTVSPETISLNVKGPGLQRMVLVDLPGVINTVTSGMAPDTKETIFSISKAYMQNPNAIILCIQDGSVDAERSIVTDLVSQMDPHGRRTIFVLTKVDLAEKNVASPSRIQQIIEGKLFPMKALGYFAVVTGKGNSSESIEAIREYEEEFFQNSKLLKTSMLKAHQVTTRNLSLAVSDCFWKMVRESVEQQADSFKATRFNLETEWKNNYPRLRELDRNELFEKAKNEILDEVISLSQVTPKHWEEILQQSLWERVSTHVIENIYLPAAQTMNSGTFNTTVDIKLKQWTDKQLPNKAVEVAWETLQEEFSRFMTEPKGKEHDDIFDKLKEAVKEESIKRHKWNDFAEDSLRVIQHNALEDRSISDKQQWDAAIYFMEEALQARLKDTENAIENMVGPDWKKRWLYWKNRTQEQCVHNETKNELEKMLKCNEEHPAYLASDEITTVRKNLESRGVEVDPSLIKDTWHQVYRRHFLKTALNHCNLCRRGFYYYQRHFVDSELECNDVVLFWRIQRMLAITANTLRQQLTNTEVRRLEKNVKEVLEDFAEDGEKKIKLLTGKRVQLAEDLKKVREIQEKLDAFIEALHQEK

SEQ ID NO: 9 - DNA, 6399 bp, Homo sapiens
gtgctgcccgcctagaaagggtgaagtggttgtttccgtgacggactgagtacgggtgcctgtcaggctcttgcggaagtccatgcgccattgggagggcctcggccgcggctctgtgcccttgctgctgagggccacttcctgggtcattcctggaccgggagccgggctggggctcacacgggggctcccgcgtggccgtctcggcgcctgcgtgacctccccgccggcgggatgtggcgactacgtcgggccgctgtggcctgtgaggtctgccagtctttagtgaaacacagctctggaataaaaggaagtttaccactacaaaaactacatctggtttcacgaagcatttatcattcacatcatcctaccttaaagcttcaacgaccccaattaaggacatcctttcagcagttctcttctctgacaaaccttcctttacgtaaactgaaattctctccaattaaatatggctaccagcctcgcaggaatttttggccagcaagattagctacgagactcttaaaacttcgctatctcatactaggatcggctgttgggggtggctacacagccaaaaagacttttgatcagtggaaagatatgataccggaccttagtgaatataaatggattgtgcctgacattgtgtgggaaattgatgagtatatcgattttgagaaaattagaaaagcccttcctagttcagaagaccttgtaaagttagcaccagactttgacaagattgttgaaagccttagcttattgaaggacttttttacctcaggtcacaaattggttagtgaagtcataggagcttctgacctacttctcttgttaggttctccggaagaaacggcgtttagagcaacagatcgtggatctgaaagtgacaagcattttagaaaggtgtcagacaaagagaaaattgaccaacttcaggaagaacttctgcacactcagttgaagtatcagagaatcttggaacgattagaaaaggagaacaaagaattgagaaaattagtattgcagaaagatgacaaaggcattcatcatagaaagcttaagaaatctttgattgacatgtattctgaagttcttgatgttctctctgattatgatgccagttataatacgcaagatcatctgccacgggttgttgtggttggagatcagagtgctggaaagactagtgtgttggaaatgattgcccaagctcgaatattcccaagaggatctggggagatgatgacacgttctccagttaaggtgactctgagtgaaggtcctcaccatgtggccctatttaaagatagttctcgggagtttgatcttaccaaagaagaagatcttgcagcattaagacatgaaatagaacttcgaatgaggaaaaatgtgaaagaaggctgtaccgttagccctgagaccatatccttaaatgtaaaaggccctggactacagaggatggtgcttgttgacttaccaggtgtgattaatactgtgacatcaggcatggctcctgacacaaaggaaactattttcagtatcagcaaagcttacatgcagaatcctaatgccatcatactgtgtattcaagatggatctgtggatgctgaacgcagtattgttacagacttggtcagtcaaatggaccctcatggaaggagaaccatattcgttttgaccaaagtagacctggcagagaaaaatgtagccagtccaagcaggattcagcagataattgaaggaaagctcttcccaatgaaagctttaggttattttgctgttgtaacaggaaaagggaacagctctgaaagcattgaagctataagagaatatgaagaagagttttttcagaattcaaagctcctaaagacaagcatgctaaaggcacaccaagtgactacaagaaatttaagccttgcagtatcagactgcttttggaaaatggtacgagagtctgttgaacaacaggctgatagtttcaaagcaacacgttttaaccttgaaactgaatggaagaataactatcctcgcctgcgggaacttgaccggaatgaactatttgaaaaagctaaaaatgaaatccttgatgaagttatcagtctgagccaggttacaccaaaacattgggaggaaatccttcaacaatctttgtgggaaagagtatcaactcatgtgattgaaaacatctaccttccagctgcgcagaccatgaattcaggaacttttaacaccacagtggatatcaagcttaaacagtggactgataaacaacttcctaataaagcagtagaggttgcttgggagaccctacaagaagaattttcccgctttatgacagaaccgaaagggaaagagcatgatgacatatttgataaacttaaagaggctgttaaggaagaaagtattaaacgacacaagtggaatgactttgcggaggacagcttgagggttattcaacacaatgctttggaagaccgatccatatctgataaacagcaatgggatgcagctatttattttatggaagaggctctgcaggctcgtctcaaggatactgaaaatgcaattgaaaacatggtgggtccagactggaaaaagaggtggttatactggaagaatcggacccaagaacagtgtgttcacaatgaaaccaagaatgaattggagaagatgttgaaatgtaatgaggagcacccagcttatcttgcaagtgatgaaataaccacagtccggaagaaccttgaatcccgaggagtagaagtagatccaagcttgattaaggatacttggcatcaagtttatagaagacattttttaaaaacagctctaaaccattgtaacctttgtcgaagaggtttttattactaccaaaggcattttgtagattctgagttggaatgcaatgatgtggtcttgttttggcgtatacagcgcatgcttgctatcaccgcaaatactttaaggcaacaacttacaaatactgaagttaggcgattagagaaaaatgttaaagaggtattggaagattttgctgaagatggtgagaagaagattaaattgcttactggtaaacgcgttcaactggcggaagacctcaagaaagttagagaaattcaagaaaaacttgatgctttcattgaagctcttcatcaggagaaataaattaaaatcgtactcataatcagctctgcatacatctgaagaacaaaaacatcaacgtcttttgtccagcctctttttcttctgctgttccacctttctaaacatacaataaagtcatgggataaaaataatcgatgtatgttacgggcgctttaaccatcagctgcctctcgaatggaagaacagtggtaatggattaacatcctattttgttgtactaaagtgacaaatcggaataatataattggtatggccattaggttcagtccttgaagataagaaacttgttctctgtttgttgtcttatttgtggtggcactcgtttaatggattaactgaggttgctcaatgttcagtttcttttccagaaatacaatgctaggtgttttgaaataaaacttatatagcaattgtttaaagttatcaattgtatataaaatcacagtagcctgctaaatcattgtatgtgtctgtagtattctattcccagaaactatttgaccatgataattcagtttatattcaccacatgaaagaaaaatgggtaacagaagaacccttaaaacaggttaatttggattgtaacgttcagtgaaagaaatttcaacccttcatagccagcgaagaaatttgccttggaagccaagtcagtaccagcttacctatttgattcagttgctgttttctcactctctatatccatttgaaattgatttattttagatgttgtatacttacgttaggctttctgttaatagtggtttttctcctgttgacagagccaccggattatgacacaggatgaggaagattaaggataatcaattgactaatttcatttagaatattatcaaacatttcaactaggtatcagaaaaaggctttctttcataagactattttaaatagaaattatttcaacaattaaagtaatgttgaccatccccctctcagctgaataaagaaaaatttagttcaatttattgcaatttaattacaatactaccttcacaacattttcatgtgttttaaataaatattttttaattggctaaaggacattcaagcaaagaaatgctttctttacttaaaatgtctatctcatttgctgccttttcactaagcctttactttgttaataaaagtgtccattgtgtgatgtttttgattttacagtttgctaaatcttattttcttggagttgctttttggtaacagccccattgctactccccattttattgttttacatcaatgcatgcttcgttgtgatccctcaagatgtaacacttggtatgctcggttgaggatatgaaaaaatacttccgaaaccaggaattcaatgtatgtttgttttatactgtttgataagaaaagtaggtccagccttaagcagcacagatgcgctggtagatgcatagtcaggaactttttttatttcttttaggtctagggacaggagtgaatagaaagggaggagagctctattatgttctatacacagattaggagatgaccttactgggtacacccctctaaccagtgcttacaggttaatgcatgttaatgaatatttttgcagttgtaaagcataacaattacaactacacatctatttctaaagaataaaacaggaccatatttatttacttctgtcaactatagaaagaaagaccttcagctgtatttccacagatttctcccaaggaaaaggctaatattagtcactactgttatcacatccctttgtataagttttaaaaagagatggagggagatcttcatttctttgaggagatcagtattgtaacgtatgtgaatagatgataacaattaatattactaaaagtcccacatgagagtcctgacgccctctccatgccccacagtaatgtggcttctttcatgggtttttttttcttctttttagctgatctcatcctaagcatgctttatttttccttgaaagctaggtatttatcaactgcagatgttattgaaagaaaataaaattcagtctcaagagtaaaccctgtgtcttgtgtctgtagttcaaaagtcagaaatgattctaatttaaacaaaaagatactaaatatacagaagttaaattcgaactagccacagaatcatttgtttttatgtcagaatttgcaaagagtggagtggacaaagctctgtatggaagactgaacaactgtaaatagatgatatccaaacttaatttggctaggacttcaattttaaaaatcagtgtacctaggcagtgcacagcacgaaataagtggcccttgcagcttccccgtttaacccactgtgctatagttgcgggtggaacagtcaacctttctagtagtttatgatattgccctctttgtattcccattttctacagttttttccgcagacttctttctgcaaattattcagcctccaaatgcaaatgaatgatataaaaataagtagggaacatggcagagagtggtgcttcccagcctcacaatgtgggaatttgacataggatgagagtcagagtataggtttaaaagataaaatctttagttaataattttgtatttatttattctagatgtatgtatctgaggaaagaaatctggtatttttgctttccaataaaggggatcaaagtaatggtttttctctcagttctctaagctggtctatgttatagctctagcagtatggaaatgtgctttaaaatatgcttaccttttgaatgatcatggctatatgttgttgagatatttgaaacttaccttgttttcacttgtgcactgtgaatgaactttgtattatttttttaaaaccttcacattacgtgtagatattattgcaacttatattttgcctgagcttgatcaaaggtcatttgtgtagatgagtaattaaaaaatatttaaatcacattataattctattattggagagcatcttttaaatttttttctgttttaacgagggaaagagaaacctgtatacctagggtcattatttgaccccatagtataaccagattcatggtctaacaagctctcagtgtggcttttctctgaatgcttgaatttcacatgccttgcatttcacagttgtactccatggtcaaccggtgctttttttcacatcgtggtacttgtcaaaacattttgttattttccttggtaaaatatataaaaaaggttttctaatttcaaaaaaaaaaaaaaaaaa

SEQ ID NO: 10 - protein, 978 aa, Homo sapiens
MWRLRRAAVACEVCQSLVKHSSGIKGSLPLQKLHLVSRSIYHSHHPTLKLQRPQLRTSFQQFSSLTNLPLRKLKFSPIKYGYQPRRNFWPARLATRLLKLRYLILGSAVGGGYTAKKTFDQWKDMIPDLSEYKWIVPDIVWEIDEYIDFEKIRKALPSSEDLVKLAPDFDKIVESLSLLKDFFTSGHKLVSEVIGASDLLLLLGSPEETAFRATDRGSESDKHFRKVSDKEKIDQLQEELLHTQLKYQRILERLEKENKELRKLVLQKDDKGIHHRKLKKSLIDMYSEVLDVLSDYDASYNTQDHLPRVVVVGDQSAGKTSVLEMIAQARIFPRGSGEMMTRSPVKVTLSEGPHHVALFKDSSREFDLTKEEDLAALRHEIELRMRKNVKEGCTVSPETISLNVKGPGLQRMVLVDLPGVINTVTSGMAPDTKETIFSISKAYMQNPNAIILCIQDGSVDAERSIVTDLVSQMDPHGRRTIFVLTKVDLAEKNVASPSRIQQIIEGKLFPMKALGYFAVVTGKGNSSESIEAIREYEEEFFQNSKLLKTSMLKAHQVTTRNLSLAVSDCFWKMVRESVEQQADSFKATRFNLETEWKNNYPRLRELDRNELFEKAKNEILDEVISLSQVTPKHWEEILQQSLWERVSTHVIENIYLPAAQTMNSGTFNTTVDIKLKQWTDKQLPNKAVEVAWETLQEEFSRFMTEPKGKEHDDIFDKLKEAVKEESIKRHKWNDFAEDSLRVIQHNALEDRSISDKQQWDAAIYFMEEALQARLKDTENAIENMVGPDWKKRWLYWKNRTQEQCVHNETKNELEKMLKCNEEHPAYLASDEITTVRKNLESRGVEVDPSLIKDTWHQVYRRHFLKTALNHCNLCRRGFYYYQRHFVDSELECNDVVLFWRIQRMLAITANTLRQQLTNTEVRRLEKNVKEVLEDFAEDGEKKIKLLTGKRVQLAEDLKKVREIQEKLDAFIEALHQEK

SEQ ID NO: 11 - DNA, 6402 bp, Homo sapiens
gtgctgcccgcctagaaagggtgaagtggttgtttccgtgacggactgagtacgggtgcctgtcaggctcttgcggaagtccatgcgccattgggagggcctcggccgcggctctgtgcccttgctgctgagggccacttcctgggtcattcctggaccgggagccgggctggggctcacacgggggctcccgcgtggccgtctcggcgcctgcgtgacctccccgccggcgggatgtggcgactacgtcgggccgctgtggcctgtgaggtctgccagtctttagtgaaacacagctctggaataaaaggaagtttaccactacaaaaactacatctggtttcacgaagcatttatcattcacatcatcctaccttaaagcttcaacgaccccaattaaggacatcctttcagcagttctcttctctgacaaaccttcctttacgtaaactgaaattctctccaattaaatatggctaccagcctcgcaggaatttttggccagcaagattagctacgagactcttaaaacttcgctatctcatactaggatcggctgttgggggtggctacacagccaaaaagacttttgatcagtggaaagatatgataccggaccttagtgaatataaatggattgtgcctgacattgtgtgggaaattgatgagtatatcgattttggtcacaaattggttagtgaagtcataggagcttctgacctacttctcttgttaggttctccggaagaaacggcgtttagagcaacagatcgtggatctgaaagtgacaagcattttagaaagggtctgcttggtgagctcattctcttacaacaacaaattcaagagcatgaagaggaagcgcgcagagccgctggccaatatagcacgagctatgcccaacagaagcgcaaggtgtcagacaaagagaaaattgaccaacttcaggaagaacttctgcacactcagttgaagtatcagagaatcttggaacgattagaaaaggagaacaaagaattgagaaaattagtattgcagaaagatgacaaaggcattcatcatagaaagcttaagaaatctttgattgacatgtattctgaagttcttgatgttctctctgattatgatgccagttataatacgcaagatcatctgccacgggttgttgtggttggagatcagagtgctggaaagactagtgtgttggaaatgattgcccaagctcgaatattcccaagaggatctggggagatgatgacacgttctccagttaaggtgactctgagtgaaggtcctcaccatgtggccctatttaaagatagttctcgggagtttgatcttaccaaagaagaagatcttgcagcattaagacatgaaatagaacttcgaatgaggaaaaatgtgaaagaaggctgtaccgttagccctgagaccatatccttaaatgtaaaaggccctggactacagaggatggtgcttgttgacttaccaggtgtgattaatactgtgacatcaggcatggctcctgacacaaaggaaactattttcagtatcagcaaagcttacatgcagaatcctaatgccatcatactgtgtattcaagatggatctgtggatgctgaacgcagtattgttacagacttggtcagtcaaatggaccctcatggaaggagaaccatattcgttttgaccaaagtagacctggcagagaaaaatgtagccagtccaagcaggattcagcagataattgaaggaaagctcttcccaatgaaagctttaggttattttgctgttgtaacaggaaaagggaacagctctgaaagcattgaagctataagagaatatgaagaagagttttttcagaattcaaagctcctaaagacaagcatgctaaaggcacaccaagtgactacaagaaatttaagccttgcagtatcagactgcttttggaaaatggtacgagagtctgttgaacaacaggctgatagtttcaaagcaacacgttttaaccttgaaactgaatggaagaataactatcctcgcctgcgggaacttgaccggaatgaactatttgaaaaagctaaaaatgaaatccttgatgaagttatcagtctgagccaggttacaccaaaacattgggaggaaatccttcaacaatctttgtgggaaagagtatcaactcatgtgattgaaaacatctaccttccagctgcgcagaccatgaattcaggaacttttaacaccacagtggatatcaagcttaaacagtggactgataaacaacttcctaataaagcagtagaggttgcttgggagaccctacaagaagaattttcccgctttatgacagaaccgaaagggaaagagcatgatgacatatttgataaacttaaagaggctgttaaggaagaaagtattaaacgacacaagtggaatgactttgcggaggacagcttgagggttattcaacacaatgctttggaagaccgatccatatctgataaacagcaatgggatgcagctatttattttatggaagaggctctgcaggctcgtctcaaggatactgaaaatgcaattgaaaacatggtgggtccagactggaaaaagaggtggttatactggaagaatcggacccaagaacagtgtgttcacaatgaaaccaagaatgaattggagaagatgttgaaatgtaatgaggagcacccagcttatcttgcaagtgatgaaataaccacagtccggaagaaccttgaatcccgaggagtagaagtagatccaagcttgattaaggatacttggcatcaagtttatagaagacattttttaaaaacagctctaaaccattgtaacctttgtcgaagaggtttttattactaccaaaggcattttgtagattctgagttggaatgcaatgatgtggtcttgttttggcgtatacagcgcatgcttgctatcaccgcaaatactttaaggcaacaacttacaaatactgaagttaggcgattagagaaaaatgttaaagaggtattggaagattttgctgaagatggtgagaagaagattaaattgcttactggtaaacgcgttcaactggcggaagacctcaagaaagttagagaaattcaagaaaaacttgatgctttcattgaagctcttcatcaggagaaataaattaaaatcgtactcataatcagctctgcatacatctgaagaacaaaaacatcaacgtcttttgtccagcctctttttcttctgctgttccacctttctaaacatacaataaagtcatgggataaaaataatcgatgtatgttacgggcgctttaaccatcagctgcctctcgaatggaagaacagtggtaatggattaacatcctattttgttgtactaaagtgacaaatcggaataatataattggtatggccattaggttcagtccttgaagataagaaacttgttctctgtttgttgtcttatttgtggtggcactcgtttaatggattaactgaggttgctcaatgttcagtttcttttccagaaatacaatgctaggtgttttgaaataaaacttatatagcaattgtttaaagttatcaattgtatataaaatcacagtagcctgctaaatcattgtatgtgtctgtagtattctattcccagaaactatttgaccatgataattcagtttatattcaccacatgaaagaaaaatgggtaacagaagaacccttaaaacaggttaatttggattgtaacgttcagtgaaagaaatttcaacccttcatagccagcgaagaaatttgccttggaagccaagtcagtaccagcttacctatttgattcagttgctgttttctcactctctatatccatttgaaattgatttattttagatgttgtatacttacgttaggctttctgttaatagtggtttttctcctgttgacagagccaccggattatgacacaggatgaggaagattaaggataatcaattgactaatttcatttagaatattatcaaacatttcaactaggtatcagaaaaaggctttctttcataagactattttaaatagaaattatttcaacaattaaagtaatgttgaccatccccctctcagctgaataaagaaaaatttagttcaatttattgcaatttaattacaatactaccttcacaacattttcatgtgttttaaataaatattttttaattggctaaaggacattcaagcaaagaaatgctttctttacttaaaatgtctatctcatttgctgccttttcactaagcctttactttgttaataaaagtgtccattgtgtgatgtttttgattttacagtttgctaaatcttattttcttggagttgctttttggtaacagccccattgctactccccattttattgttttacatcaatgcatgcttcgttgtgatccctcaagatgtaacacttggtatgctcggttgaggatatgaaaaaatacttccgaaaccaggaattcaatgtatgtttgttttatactgtttgataagaaaagtaggtccagccttaagcagcacagatgcgctggtagatgcatagtcaggaactttttttatttcttttaggtctagggacaggagtgaatagaaagggaggagagctctattatgttctatacacagattaggagatgaccttactgggtacacccctctaaccagtgcttacaggttaatgcatgttaatgaatatttttgcagttgtaaagcataacaattacaactacacatctatttctaaagaataaaacaggaccatatttatttacttctgtcaactatagaaagaaagaccttcagctgtatttccacagatttctcccaaggaaaaggctaatattagtcactactgttatcacatccctttgtataagttttaaaaagagatggagggagatcttcatttctttgaggagatcagtattgtaacgtatgtgaatagatgataacaattaatattactaaaagtcccacatgagagtcctgacgccctctccatgccccacagtaatgtggcttctttcatgggtttttttttcttctttttagctgatctcatcctaagcatgctttatttttccttgaaagctaggtatttatcaactgcagatgttattgaaagaaaataaaattcagtctcaagagtaaaccctgtgtcttgtgtctgtagttcaaaagtcagaaatgattctaatttaaacaaaaagatactaaatatacagaagttaaattcgaactagccacagaatcatttgtttttatgtcagaatttgcaaagagtggagtggacaaagctctgtatggaagactgaacaactgtaaatagatgatatccaaacttaatttggctaggacttcaattttaaaaatcagtgtacctaggcagtgcacagcacgaaataagtggcccttgcagcttccccgtttaacccactgtgctatagttgcgggtggaacagtcaacctttctagtagtttatgatattgccctctttgtattcccattttctacagttttttccgcagacttctttctgcaaattattcagcctccaaatgcaaatgaatgatataaaaataagtagggaacatggcagagagtggtgcttcccagcctcacaatgtgggaatttgacataggatgagagtcagagtataggtttaaaagataaaatctttagttaataattttgtatttatttattctagatgtatgtatctgaggaaagaaatctggtatttttgctttccaataaaggggatcaaagtaatggtttttctctcagttctctaagctggtctatgttatagctctagcagtatggaaatgtgctttaaaatatgcttaccttttgaatgatcatggctatatgttgttgagatatttgaaacttaccttgttttcacttgtgcactgtgaatgaactttgtattatttttttaaaaccttcacattacgtgtagatattattgcaacttatattttgcctgagcttgatcaaaggtcatttgtgtagatgagtaattaaaaaatatttaaatcacattataattctattattggagagcatcttttaaatttttttctgttttaacgagggaaagagaaacctgtatacctagggtcattatttgaccccatagtataaccagattcatggtctaacaagctctcagtgtggcttttctctgaatgcttgaatttcacatgccttgcatttcacagttgtactccatggtcaaccggtgctttttttcacatcgtggtacttgtcaaaacattttgttattttccttggtaaaatatataaaaaaggttttctaatttcaaaaaaaaaaaaaaaaaa

SEQ ID NO: 12 - protein, 979 aa, Homo sapiens
MWRLRRAAVACEVCQSLVKHSSGIKGSLPLQKLHLVSRSIYHSHHPTLKLQRPQLRTSFQQFSSLTNLPLRKLKFSPIKYGYQPRRNFWPARLATRLLKLRYLILGSAVGGGYTAKKTFDQWKDMIPDLSEYKWIVPDIVWEIDEYIDFGHKLVSEVIGASDLLLLLGSPEETAFRATDRGSESDKHFRKGLLGELILLQQQIQEHEEEARRAAGQYSTSYAQQKRKVSDKEKIDQLQEELLHTQLKYQRILERLEKENKELRKLVLQKDDKGIHHRKLKKSLIDMYSEVLDVLSDYDASYNTQDHLPRVVVVGDQSAGKTSVLEMIAQARIFPRGSGEMMTRSPVKVTLSEGPHHVALFKDSSREFDLTKEEDLAALRHEIELRMRKNVKEGCTVSPETISLNVKGPGLQRMVLVDLPGVINTVTSGMAPDTKETIFSISKAYMQNPNAIILCIQDGSVDAERSIVTDLVSQMDPHGRRTIFVLTKVDLAEKNVASPSRIQQIIEGKLFPMKALGYFAVVTGKGNSSESIEAIREYEEEFFQNSKLLKTSMLKAHQVTTRNLSLAVSDCFWKMVRESVEQQADSFKATRFNLETEWKNNYPRLRELDRNELFEKAKNEILDEVISLSQVTPKHWEEILQQSLWERVSTHVIENIYLPAAQTMNSGTFNTTVDIKLKQWTDKQLPNKAVEVAWETLQEEFSRFMTEPKGKEHDDIFDKLKEAVKEESIKRHKWNDFAEDSLRVIQHNALEDRSISDKQQWDAAIYFMEEALQARLKDTENAIENMVGPDWKKRWLYWKNRTQEQCVHNETKNELEKMLKCNEEHPAYLASDEITTVRKNLESRGVEVDPSLIKDTWHQVYRRHFLKTALNHCNLCRRGFYYYQRHFVDSELECNDVVLFWRIQRMLAITANTLRQQLTNTEVRRLEKNVKEVLEDFAEDGEKKIKLLTGKRVQLAEDLKKVREIQEKLDAFIEALHQEK

SEQ ID NO: 13 - DNA, 6456 bp, Homo sapiens
gtgctgcccgcctagaaagggtgaagtggttgtttccgtgacggactgagtacgggtgcctgtcaggctcttgcggaagtccatgcgccattgggagggcctcggccgcggctctgtgcccttgctgctgagggccacttcctgggtcattcctggaccgggagccgggctggggctcacacgggggctcccgcgtggccgtctcggcgcctgcgtgacctccccgccggcgggatgtggcgactacgtcgggccgctgtggcctgtgaggtctgccagtctttagtgaaacacagctctggaataaaaggaagtttaccactacaaaaactacatctggtttcacgaagcatttatcattcacatcatcctaccttaaagcttcaacgaccccaattaaggacatcctttcagcagttctcttctctgacaaaccttcctttacgtaaactgaaattctctccaattaaatatggctaccagcctcgcaggaatttttggccagcaagattagctacgagactcttaaaacttcgctatctcatactaggatcggctgttgggggtggctacacagccaaaaagacttttgatcagtggaaagatatgataccggaccttagtgaatataaatggattgtgcctgacattgtgtgggaaattgatgagtatatcgattttgagaaaattagaaaagcccttcctagttcagaagaccttgtaaagttagcaccagactttgacaagattgttgaaagccttagcttattgaaggacttttttacctcaggttctccggaagaaacggcgtttagagcaacagatcgtggatctgaaagtgacaagcattttagaaagggtctgcttggtgagctcattctcttacaacaacaaattcaagagcatgaagaggaagcgcgcagagccgctggccaatatagcacgagctatgcccaacagaagcgcaaggtgtcagacaaagagaaaattgaccaacttcaggaagaacttctgcacactcagttgaagtatcagagaatcttggaacgattagaaaaggagaacaaagaattgagaaaattagtattgcagaaagatgacaaaggcattcatcatagaaagcttaagaaatctttgattgacatgtattctgaagttcttgatgttctctctgattatgatgccagttataatacgcaagatcatctgccacgggttgttgtggttggagatcagagtgctggaaagactagtgtgttggaaatgattgcccaagctcgaatattcccaagaggatctggggagatgatgacacgttctccagttaaggtgactctgagtgaaggtcctcaccatgtggccctatttaaagatagttctcgggagtttgatcttaccaaagaagaagatcttgcagcattaagacatgaaatagaacttcgaatgaggaaaaatgtgaaagaaggctgtaccgttagccctgagaccatatccttaaatgtaaaaggccctggactacagaggatggtgcttgttgacttaccaggtgtgattaatactgtgacatcaggcatggctcctgacacaaaggaaactattttcagtatcagcaaagcttacatgcagaatcctaatgccatcatactgtgtattcaagatggatctgtggatgctgaacgcagtattgttacagacttggtcagtcaaatggaccctcatggaaggagaaccatattcgttttgaccaaagtagacctggcagagaaaaatgtagccagtccaagcaggattcagcagataattgaaggaaagctcttcccaatgaaagctttaggttattttgctgttgtaacaggaaaagggaacagctctgaaagcattgaagctataagagaatatgaagaagagttttttcagaattcaaagctcctaaagacaagcatgctaaaggcacaccaagtgactacaagaaatttaagccttgcagtatcagactgcttttggaaaatggtacgagagtctgttgaacaacaggctgatagtttcaaagcaacacgttttaaccttgaaactgaatggaagaataactatcctcgcctgcgggaacttgaccggaatgaactatttgaaaaagctaaaaatgaaatccttgatgaagttatcagtctgagccaggttacaccaaaacattgggaggaaatccttcaacaatctttgtgggaaagagtatcaactcatgtgattgaaaacatctaccttccagctgcgcagaccatgaattcaggaacttttaacaccacagtggatatcaagcttaaacagtggactgataaacaacttcctaataaagcagtagaggttgcttgggagaccctacaagaagaattttcccgctttatgacagaaccgaaagggaaagagcatgatgacatatttgataaacttaaagaggctgttaaggaagaaagtattaaacgacacaagtggaatgactttgcggaggacagcttgagggttattcaacacaatgctttggaagaccgatccatatctgataaacagcaatgggatgcagctatttattttatggaagaggctctgcaggctcgtctcaaggatactgaaaatgcaattgaaaacatggtgggtccagactggaaaaagaggtggttatactggaagaatcggacccaagaacagtgtgttcacaatgaaaccaagaatgaattggagaagatgttgaaatgtaatgaggagcacccagcttatcttgcaagtgatgaaataaccacagtccggaagaaccttgaatcccgaggagtagaagtagatccaagcttgattaaggatacttggcatcaagtttatagaagacattttttaaaaacagctctaaaccattgtaacctttgtcgaagaggtttttattactaccaaaggcattttgtagattctgagttggaatgcaatgatgtggtcttgttttggcgtatacagcgcatgcttgctatcaccgcaaatactttaaggcaacaacttacaaatactgaagttaggcgattagagaaaaatgttaaagaggtattggaagattttgctgaagatggtgagaagaagattaaattgcttactggtaaacgcgttcaactggcggaagacctcaagaaagttagagaaattcaagaaaaacttgatgctttcattgaagctcttcatcaggagaaataaattaaaatcgtactcataatcagctctgcatacatctgaagaacaaaaacatcaacgtcttttgtccagcctctttttcttctgctgttccacctttctaaacatacaataaagtcatgggataaaaataatcgatgtatgttacgggcgctttaaccatcagctgcctctcgaatggaagaacagtggtaatggattaacatcctattttgttgtactaaagtgacaaatcggaataatataattggtatggccattaggttcagtccttgaagataagaaacttgttctctgtttgttgtcttatttgtggtggcactcgtttaatggattaactgaggttgctcaatgttcagtttcttttccagaaatacaatgctaggtgttttgaaataaaacttatatagcaattgtttaaagttatcaattgtatataaaatcacagtagcctgctaaatcattgtatgtgtctgtagtattctattcccagaaactatttgaccatgataattcagtttatattcaccacatgaaagaaaaatgggtaacagaagaacccttaaaacaggttaatttggattgtaacgttcagtgaaagaaatttcaacccttcatagccagcgaagaaatttgccttggaagccaagtcagtaccagcttacctatttgattcagttgctgttttctcactctctatatccatttgaaattgatttattttagatgttgtatacttacgttaggctttctgttaatagtggtttttctcctgttgacagagccaccggattatgacacaggatgaggaagattaaggataatcaattgactaatttcatttagaatattatcaaacatttcaactaggtatcagaaaaaggctttctttcataagactattttaaatagaaattatttcaacaattaaagtaatgttgaccatccccctctcagctgaataaagaaaaatttagttcaatttattgcaatttaattacaatactaccttcacaacattttcatgtgttttaaataaatattttttaattggctaaaggacattcaagcaaagaaatgctttctttacttaaaatgtctatctcatttgctgccttttcactaagcctttactttgttaataaaagtgtccattgtgtgatgtttttgattttacagtttgctaaatcttattttcttggagttgctttttggtaacagccccattgctactccccattttattgttttacatcaatgcatgcttcgttgtgatccctcaagatgtaacacttggtatgctcggttgaggatatgaaaaaatacttccgaaaccaggaattcaatgtatgtttgttttatactgtttgataagaaaagtaggtccagccttaagcagcacagatgcgctggtagatgcatagtcaggaactttttttatttcttttaggtctagggacaggagtgaatagaaagggaggagagctctattatgttctatacacagattaggagatgaccttactgggtacacccctctaaccagtgcttacaggttaatgcatgttaatgaatatttttgcagttgtaaagcataacaattacaactacacatctatttctaaagaataaaacaggaccatatttatttacttctgtcaactatagaaagaaagaccttcagctgtatttccacagatttctcccaaggaaaaggctaatattagtcactactgttatcacatccctttgtataagttttaaaaagagatggagggagatcttcatttctttgaggagatcagtattgtaacgtatgtgaatagatgataacaattaatattactaaaagtcccacatgagagtcctgacgccctctccatgccccacagtaatgtggcttctttcatgggtttttttttcttctttttagctgatctcatcctaagcatgctttatttttccttgaaagctaggtatttatcaactgcagatgttattgaaagaaaataaaattcagtctcaagagtaaaccctgtgtcttgtgtctgtagttcaaaagtcagaaatgattctaatttaaacaaaaagatactaaatatacagaagttaaattcgaactagccacagaatcatttgtttttatgtcagaatttgcaaagagtggagtggacaaagctctgtatggaagactgaacaactgtaaatagatgatatccaaacttaatttggctaggacttcaattttaaaaatcagtgtacctaggcagtgcacagcacgaaataagtggcccttgcagcttccccgtttaacccactgtgctatagttgcgggtggaacagtcaacctttctagtagtttatgatattgccctctttgtattcccattttctacagttttttccgcagacttctttctgcaaattattcagcctccaaatgcaaatgaatgatataaaaataagtagggaacatggcagagagtggtgcttcccagcctcacaatgtgggaatttgacataggatgagagtcagagtataggtttaaaagataaaatctttagttaataattttgtatttatttattctagatgtatgtatctgaggaaagaaatctggtatttttgctttccaataaaggggatcaaagtaatggtttttctctcagttctctaagctggtctatgttatagctctagcagtatggaaatgtgctttaaaatatgcttaccttttgaatgatcatggctatatgttgttgagatatttgaaacttaccttgttttcacttgtgcactgtgaatgaactttgtattatttttttaaaaccttcacattacgtgtagatattattgcaacttatattttgcctgagcttgatcaaaggtcatttgtgtagatgagtaattaaaaaatatttaaatcacattataattctattattggagagcatcttttaaatttttttctgttttaacgagggaaagagaaacctgtatacctagggtcattatttgaccccatagtataaccagattcatggtctaacaagctctcagtgtggcttttctctgaatgcttgaatttcacatgccttgcatttcacagttgtactccatggtcaaccggtgctttttttcacatcgtggtacttgtcaaaacattttgttattttccttggtaaaatatataaaaaaggttttctaatttcaaaaaaaaaaaaaaaaaa

SEQ ID NO: 14 - protein, 997 aa, Homo sapiens
MWRLRRAAVACEVCQSLVKHSSGIKGSLPLQKLHLVSRSIYHSHHPTLKLQRPQLRTSFQQFSSLTNLPLRKLKFSPIKYGYQPRRNFWPARLATRLLKLRYLILGSAVGGGYTAKKTFDQWKDMIPDLSEYKWIVPDIVWEIDEYIDFEKIRKALPSSEDLVKLAPDFDKIVESLSLLKDFFTSGSPEETAFRATDRGSESDKHFRKGLLGELILLQQQIQEHEEEARRAAGQYSTSYAQQKRKVSDKEKIDQLQEELLHTQLKYQRILERLEKENKELRKLVLQKDDKGIHHRKLKKSLIDMYSEVLDVLSDYDASYNTQDHLPRVVVVGDQSAGKTSVLEMIAQARIFPRGSGEMMTRSPVKVTLSEGPHHVALFKDSSREFDLTKEEDLAALRHEIELRMRKNVKEGCTVSPETISLNVKGPGLQRMVLVDLPGVINTVTSGMAPDTKETIFSISKAYMQNPNAIILCIQDGSVDAERSIVTDLVSQMDPHGRRTIFVLTKVDLAEKNVASPSRIQQIIEGKLFPMKALGYFAVVTGKGNSSESIEAIREYEEEFFQNSKLLKTSMLKAHQVTTRNLSLAVSDCFWKMVRESVEQQADSFKATRFNLETEWKNNYPRLRELDRNELFEKAKNEILDEVISLSQVTPKHWEEILQQSLWERVSTHVIENIYLPAAQTMNSGTFNTTVDIKLKQWTDKQLPNKAVEVAWETLQEEFSRFMTEPKGKEHDDIFDKLKEAVKEESIKRHKWNDFAEDSLRVIQHNALEDRSISDKQQWDAAIYFMEEALQARLKDTENAIENMVGPDWKKRWLYWKNRTQEQCVHNETKNELEKMLKCNEEHPAYLASDEITTVRKNLESRGVEVDPSLIKDTWHQVYRRHFLKTALNHCNLCRRGFYYYQRHFVDSELECNDVVLFWRIQRMLAITANTLRQQLTNTEVRRLEKNVKEVLEDFAEDGEKKIKLLTGKRVQLAEDLKKVREIQEKLDAFIEALHQEK

SEQ ID NO: 15 - DNA, 6510 bp, Homo sapiens
gtgctgcccgcctagaaagggtgaagtggttgtttccgtgacggactgagtacgggtgcctgtcaggctcttgcggaagtccatgcgccattgggagggcctcggccgcggctctgtgcccttgctgctgagggccacttcctgggtcattcctggaccgggagccgggctggggctcacacgggggctcccgcgtggccgtctcggcgcctgcgtgacctccccgccggcgggatgtggcgactacgtcgggccgctgtggcctgtgaggtctgccagtctttagtgaaacacagctctggaataaaaggaagtttaccactacaaaaactacatctggtttcacgaagcatttatcattcacatcatcctaccttaaagcttcaacgaccccaattaaggacatcctttcagcagttctcttctctgacaaaccttcctttacgtaaactgaaattctctccaattaaatatggctaccagcctcgcaggaatttttggccagcaagattagctacgagactcttaaaacttcgctatctcatactaggatcggctgttgggggtggctacacagccaaaaagacttttgatcagtggaaagatatgataccggaccttagtgaatataaatggattgtgcctgacattgtgtgggaaattgatgagtatatcgattttgagaaaattagaaaagcccttcctagttcagaagaccttgtaaagttagcaccagactttgacaagattgttgaaagccttagcttattgaaggacttttttacctcaggtcacaaattggttagtgaagtcataggagcttctgacctacttctcttgttaggttctccggaagaaacggcgtttagagcaacagatcgtggatctgaaagtgacaagcattttagaaagggtctgcttggtgagctcattctcttacaacaacaaattcaagagcatgaagaggaagcgcgcagagccgctggccaatatagcacgagctatgcccaacagaagcgcaaggtgtcagacaaagagaaaattgaccaacttcaggaagaacttctgcacactcagttgaagtatcagagaatcttggaacgattagaaaaggagaacaaagaattgagaaaattagtattgcagaaagatgacaaaggcattcatcatagaaagcttaagaaatctttgattgacatgtattctgaagttcttgatgttctctctgattatgatgccagttataatacgcaagatcatctgccacgggttgttgtggttggagatcagagtgctggaaagactagtgtgttggaaatgattgcccaagctcgaatattcccaagaggatctggggagatgatgacacgttctccagttaaggtgactctgagtgaaggtcctcaccatgtggccctatttaaagatagttctcgggagtttgatcttaccaaagaagaagatcttgcagcattaagacatgaaatagaacttcgaatgaggaaaaatgtgaaagaaggctgtaccgttagccctgagaccatatccttaaatgtaaaaggccctggactacagaggatggtgcttgttgacttaccaggtgtgattaatactgtgacatcaggcatggctcctgacacaaaggaaactattttcagtatcagcaaagcttacatgcagaatcctaatgccatcatactgtgtattcaagatggatctgtggatgctgaacgcagtattgttacagacttggtcagtcaaatggaccctcatggaaggagaaccatattcgttttgaccaaagtagacctggcagagaaaaatgtagccagtccaagcaggattcagcagataattgaaggaaagctcttcccaatgaaagctttaggttattttgctgttgtaacaggaaaagggaacagctctgaaagcattgaagctataagagaatatgaagaagagttttttcagaattcaaagctcctaaagacaagcatgctaaaggcacaccaagtgactacaagaaatttaagccttgcagtatcagactgcttttggaaaatggtacgagagtctgttgaacaacaggctgatagtttcaaagcaacacgttttaaccttgaaactgaatggaagaataactatcctcgcctgcgggaacttgaccggaatgaactatttgaaaaagctaaaaatgaaatccttgatgaagttatcagtctgagccaggttacaccaaaacattgggaggaaatccttcaacaatctttgtgggaaagagtatcaactcatgtgattgaaaacatctaccttccagctgcgcagaccatgaattcaggaacttttaacaccacagtggatatcaagcttaaacagtggactgataaacaacttcctaataaagcagtagaggttgcttgggagaccctacaagaagaattttcccgctttatgacagaaccgaaagggaaagagcatgatgacatatttgataaacttaaagaggctgttaaggaagaaagtattaaacgacacaagtggaatgactttgcggaggacagcttgagggttattcaacacaatgctttggaagaccgatccatatctgataaacagcaatgggatgcagctatttattttatggaagaggctctgcaggctcgtctcaaggatactgaaaatgcaattgaaaacatggtgggtccagactggaaaaagaggtggttatactggaagaatcggacccaagaacagtgtgttcacaatgaaaccaagaatgaattggagaagatgttgaaatgtaatgaggagcacccagcttatcttgcaagtgatgaaataaccacagtccggaagaaccttgaatcccgaggagtagaagtagatccaagcttgattaaggatacttggcatcaagtttatagaagacattttttaaaaacagctctaaaccattgtaacctttgtcgaagaggtttttattactaccaaaggcattttgtagattctgagttggaatgcaatgatgtggtcttgttttggcgtatacagcgcatgcttgctatcaccgcaaatactttaaggcaacaacttacaaatactgaagttaggcgattagagaaaaatgttaaagaggtattggaagattttgctgaagatggtgagaagaagattaaattgcttactggtaaacgcgttcaactggcggaagacctcaagaaagttagagaaattcaagaaaaacttgatgctttcattgaagctcttcatcaggagaaataaattaaaatcgtactcataatcagctctgcatacatctgaagaacaaaaacatcaacgtcttttgtccagcctctttttcttctgctgttccacctttctaaacatacaataaagtcatgggataaaaataatcgatgtatgttacgggcgctttaaccatcagctgcctctcgaatggaagaacagtggtaatggattaacatcctattttgttgtactaaagtgacaaatcggaataatataattggtatggccattaggttcagtccttgaagataagaaacttgttctctgtttgttgtcttatttgtggtggcactcgtttaatggattaactgaggttgctcaatgttcagtttcttttccagaaatacaatgctaggtgttttgaaataaaacttatatagcaattgtttaaagttatcaattgtatataaaatcacagtagcctgctaaatcattgtatgtgtctgtagtattctattcccagaaactatttgaccatgataattcagtttatattcaccacatgaaagaaaaatgggtaacagaagaacccttaaaacaggttaatttggattgtaacgttcagtgaaagaaatttcaacccttcatagccagcgaagaaatttgccttggaagccaagtcagtaccagcttacctatttgattcagttgctgttttctcactctctatatccatttgaaattgatttattttagatgttgtatacttacgttaggctttctgttaatagtggtttttctcctgttgacagagccaccggattatgacacaggatgaggaagattaaggataatcaattgactaatttcatttagaatattatcaaacatttcaactaggtatcagaaaaaggctttctttcataagactattttaaatagaaattatttcaacaattaaagtaatgttgaccatccccctctcagctgaataaagaaaaatttagttcaatttattgcaatttaattacaatactaccttcacaacattttcatgtgttttaaataaatattttttaattggctaaaggacattcaagcaaagaaatgctttctttacttaaaatgtctatctcatttgctgccttttcactaagcctttactttgttaataaaagtgtccattgtgtgatgtttttgattttacagtttgctaaatcttattttcttggagttgctttttggtaacagccccattgctactccccattttattgttttacatcaatgcatgcttcgttgtgatccctcaagatgtaacacttggtatgctcggttgaggatatgaaaaaatacttccgaaaccaggaattcaatgtatgtttgttttatactgtttgataagaaaagtaggtccagccttaagcagcacagatgcgctggtagatgcatagtcaggaactttttttatttcttttaggtctagggacaggagtgaatagaaagggaggagagctctattatgttctatacacagattaggagatgaccttactgggtacacccctctaaccagtgcttacaggttaatgcatgttaatgaatatttttgcagttgtaaagcataacaattacaactacacatctatttctaaagaataaaacaggaccatatttatttacttctgtcaactatagaaagaaagaccttcagctgtatttccacagatttctcccaaggaaaaggctaatattagtcactactgttatcacatccctttgtataagttttaaaaagagatggagggagatcttcatttctttgaggagatcagtattgtaacgtatgtgaatagatgataacaattaatattactaaaagtcccacatgagagtcctgacgccctctccatgccccacagtaatgtggcttctttcatgggtttttttttcttctttttagctgatctcatcctaagcatgctttatttttccttgaaagctaggtatttatcaactgcagatgttattgaaagaaaataaaattcagtctcaagagtaaaccctgtgtcttgtgtctgtagttcaaaagtcagaaatgattctaatttaaacaaaaagatactaaatatacagaagttaaattcgaactagccacagaatcatttgtttttatgtcagaatttgcaaagagtggagtggacaaagctctgtatggaagactgaacaactgtaaatagatgatatccaaacttaatttggctaggacttcaattttaaaaatcagtgtacctaggcagtgcacagcacgaaataagtggcccttgcagcttccccgtttaacccactgtgctatagttgcgggtggaacagtcaacctttctagtagtttatgatattgccctctttgtattcccattttctacagttttttccgcagacttctttctgcaaattattcagcctccaaatgcaaatgaatgatataaaaataagtagggaacatggcagagagtggtgcttcccagcctcacaatgtgggaatttgacataggatgagagtcagagtataggtttaaaagataaaatctttagttaataattttgtatttatttattctagatgtatgtatctgaggaaagaaatctggtatttttgctttccaataaaggggatcaaagtaatggtttttctctcagttctctaagctggtctatgttatagctctagcagtatggaaatgtgctttaaaatatgcttaccttttgaatgatcatggctatatgttgttgagatatttgaaacttaccttgttttcacttgtgcactgtgaatgaactttgtattatttttttaaaaccttcacattacgtgtagatattattgcaacttatattttgcctgagcttgatcaaaggtcatttgtgtagatgagtaattaaaaaatatttaaatcacattataattctattattggagagcatcttttaaatttttttctgttttaacgagggaaagagaaacctgtatacctagggtcattatttgaccccatagtataaccagattcatggtctaacaagctctcagtgtggcttttctctgaatgcttgaatttcacatgccttgcatttcacagttgtactccatggtcaaccggtgctttttttcacatcgtggtacttgtcaaaacattttgttattttccttggtaaaatatataaaaaaggttttctaatttcaaaaaaaaaaaaaaaaaa

SEQ ID NO: 16 - protein, 1015 aa, Homo sapiens
MWRLRRAAVACEVCQSLVKHSSGIKGSLPLQKLHLVSRSIYHSHHPTLKLQRPQLRTSFQQFSSLTNLPLRKLKFSPIKYGYQPRRNFWPARLATRLLKLRYLILGSAVGGGYTAKKTFDQWKDMIPDLSEYKWIVPDIVWEIDEYIDFEKIRKALPSSEDLVKLAPDFDKIVESLSLLKDFFTSGHKLVSEVIGASDLLLLLGSPEETAFRATDRGSESDKHFRKGLLGELILLQQQIQEHEEEARRAAGQYSTSYAQQKRKVSDKEKIDQLQEELLHTQLKYQRILERLEKENKELRKLVLQKDDKGIHHRKLKKSLIDMYSEVLDVLSDYDASYNTQDHLPRVVVVGDQSAGKTSVLEMIAQARIFPRGSGEMMTRSPVKVTLSEGPHHVALFKDSSREFDLTKEEDLAALRHEIELRMRKNVKEGCTVSPETISLNVKGPGLQRMVLVDLPGVINTVTSGMAPDTKETIFSISKAYMQNPNAIILCIQDGSVDAERSIVTDLVSQMDPHGRRTIFVLTKVDLAEKNVASPSRIQQIIEGKLFPMKALGYFAVVTGKGNSSESIEAIREYEEEFFQNSKLLKTSMLKAHQVTTRNLSLAVSDCFWKMVRESVEQQADSFKATRFNLETEWKNNYPRLRELDRNELFEKAKNEILDEVISLSQVTPKHWEEILQQSLWERVSTHVIENIYLPAAQTMNSGTFNTTVDIKLKQWTDKQLPNKAVEVAWETLQEEFSRFMTEPKGKEHDDIFDKLKEAVKEESIKRHKWNDFAEDSLRVIQHNALEDRSISDKQQWDAAIYFMEEALQARLKDTENAIENMVGPDWKKRWLYWKNRTQEQCVHNETKNELEKMLKCNEEHPAYLASDEITTVRKNLESRGVEVDPSLIKDTWHQVYRRHFLKTALNHCNLCRRGFYYYQRHFVDSELECNDVVLFWRIQRMLAITANTLRQQLTNTEVRRLEKNVKEVLEDFAEDGEKKIKLLTGKRVQLAEDLKKVREIQEKLDAFIEALHQEK

SEQ ID NO: 17 - DNA, 1953 bp, Homo sapiens
gcgaagggcgccccggccggtatggcgggcaggaagtgcgggtgcgcgcctgcgcataggtcgggtctgcggtgtcaccgctttcgcttctgcttgagtaatcaagtgaaaaaatgagcttcatctgtggattgcagtctgctgctagaaaccatgttttcttccgatttaattcactgtctaactggagaaaatgtaacacattagcatccacctcacggggctgtcatcaagtacaagttaaccatatagtaaataagtatcagggactgggagtaaatcagtgtgacaggtggagttttctgcctggaaactttcatttttatagtacttttaacaacaaaagaacaggaggcctctcaagtaccaaaagtaaggaaatttggaggattaccagcaaatgtactgtatggaatgatgctttttcaagacagctgctaataaaagaagttacagcagtccctagtctgtcagtattgcatcctctaagccctgcttccataagagctattaggaatttccatacttctccacggtttcaagctgctccggttcctctcttgttgatgattcttaaaccagtacagaagttatttgcaatcattgtaggcaggggcataaggaaatggtggcaggcacttcctcctaacaagaaggaagtagttaaagaaaatataaggaagaataaatggaagctattccttggtttgagtagttttggattgctctttgtggtgttttattttactcacctggaagtaagtccaatcacaggaaggagcaagctactattattggggaaagaacagttcagacttttatcggaactggaatatgaagcatggatggaagaatttaaaaatgatatgctaactgagaaagatgcccgatacctggctgttaaagaagtgctttgtcatctaattgaatgcaataaagatgttccagggatctctcagatcaattgggttattcatgtggttgattccccaattattaatgccttcgtgcttccaaatggacaaatgtttgttttcactggatttttaaatagtgtaaccgatattcatcaactttctttccttctgggccatgaaatagcacatgcagtacttgggcatgctgcagaaaaggctggcatggttcatttgttggatttcctaggtatgattttcctcacaatgatttgggccatttgtcctcgagatagcttggcacttttgtgccagtggatacagtctaaattgcaggagtatatgtttaatagaccatacagcagaaaattggaggccgaagctgacaaaattggactactgcttgctgcaaaggcttgtgcagacataagagccagttcagtgttttggcagcaaatggagttcgttgatagcctgcatggccaacccaagatgccagaatggttatctacacacccttctcatggcaatcgagttgagtacttggatagacttatacctcaggctctcaaaattagagagatgtgtaattgtccaccactgtctaatccagaccctcgattactattcaaactcagcacgaagcattttcttgaagaatcagagaaagaagacctaaatatcacgaagaaacagaaaatggatactcttcctattcaaaaacaggagcaaataccattaacatacatagttgagaaaagaacgggcagttgaattaaaatttatgagacacaagatatatgaagaatgttgcagtccttatcattttatgttactttttaaaaaatgatgtttgaagtgaaaaaaaaaaggatattcagggtcaaatcatgtacattacagatattatctaaattcttctagaatttatttttcatgaaatattgatgtattttaatctatgttaaaatatcttcaatgaggaaaatgtcacagaataaatttatattacacattttaaaaaaaaaaaaaaaaaaaa

SEQ ID NO: 18 - protein, 524 aa, Homo sapiens
MSFICGLQSAARNHVFFRFNSLSNWRKCNTLASTSRGCHQVQVNHIVNKYQGLGVNQCDRWSFLPGNFHFYSTFNNKRTGGLSSTKSKEIWRITSKCTVWNDAFSRQLLIKEVTAVPSLSVLHPLSPASIRAIRNFHTSPRFQAAPVPLLLMILKPVQKLFAIIVGRGIRKWWQALPPNKKEVVKENIRKNKWKLFLGLSSFGLLFVVFYFTHLEVSPITGRSKLLLLGKEQFRLLSELEYEAWMEEFKNDMLTEKDARYLAVKEVLCHLIECNKDVPGISQINWVIHVVDSPIINAFVLPNGQMFVFTGFLNSVTDIHQLSFLLGHEIAHAVLGHAAEKAGMVHLLDFLGMIFLTMIWAICPRDSLALLCQWIQSKLQEYMFNRPYSRKLEAEADKIGLLLAAKACADIRASSVFWQQMEFVDSLHGQPKMPEWLSTHPSHGNRVEYLDRLIPQALKIREMCNCPPLSNPDPRLLFKLSTKHFLEESEKEDLNITKKQKMDTLPIQKQEQIPLTYIVEKRTGS

SEQ ID NO: 19 - DNA, 2952 bp, Homo sapiens
gctctaggtaagcgaaacaagccgggggactgcgagccagggactcgggccgcggggcgggaagaagtggggcagcgcttggccaggccgaaaggactttgggggtgggggctgggagtccgtgtctcgaatgagggaggagaggtggagttgccggggctcaggcccggcctcgagcatgggcggatgagaggagtcgggagccgaggcctagggtccttcgggtgaggggagacggagccagcgaggagatggagcagaagcttgtggaggagattcttcaagcaatcactatgtcaacagacacaggtgtttcccttccttcatatgaggaagatcagggatcaaaactcattcgaaaagctaaagaggcaccattcgtacccgttggaatagcgggttttgcagcaattgttgcatatggattatataaactgaagagcaggggaaatactaaaatgtccattcatctgatccacatgcgtgtggcagcccaaggctttgttgtaggagcaatgactgttggtatgggctattccatgtatcgggaattctgggcaaaacctaagccttagaagaagagatgctgtcttggtcttgttggaggagcttgctttagttagatgtcttattattaaagttacctattattgttggaaataaactaatttgtatgggtttagatggtaacatggcattttgaatattggcttcctttcttgcaggcttgatttgcttggtgaccgaattactagtgactagtttactaactaggtcattcaaggaagtcaagttaacttaaacatgtcacctaaatgcacttgatggtgttgaaatgtccaccttcttaaatttttaagatgaacttagttctaaagaagataacaggccaatcctgaaggtactccctgtttgctgcagaatgtcagatattttggatgttgcataagagtcctatttgccccagttaattcaacttttgtctgcctgttttgtggactggctggctctgttagaactctgtccaaaaagtgcatggaatataacttgtaaagcttcccacaattgacaatatatatgcatgtgtttaaaccaaatccagaaagcttaaacaatagagctgcataatagtatttattaaagaatcacaactgtaaacatgagaataatttaaggattctagtttagttttttgtaattgcaaattatatttttgctgctgatatattagaataatttttaaatgtcatcttgaaatagaaatatgtattttaagcactcacgcaaaggtaaatgaacacgttttaaatgtgtgtgttgctaattttttccataagaattgtaaacattgaactgaacaaattacctataatggatttggttaatgacttatgagcaagctggtttggccagacagtatacccaaacttttatataatatacagaaggctatcacacttgtgaaattctcttgtctaatctgaatttgcattccatggtgttaacatggtatatgtattgttattaaagtaagtgacccatgtcaaatgtcttttatttatttcatgaggaaaagctttctgtagaggaacaaatttgagaacaagtttcaggaaattgtcttttttgttgttgttctctaatcatgttctcctttctgtttcaacgattttaaaaatattttactttatggtatgttttattttttttccttttgtgggtaatttttgttctattgattatccatataaattttttttttttttttttgagacggagttattctctgtcatcttggctggcgtgcagtggcacgatcttggctcactgcaacttccatcccccaggttcaagtgattctcttgcctcagcctcctgagtagctgtgattacaggcatgcaccaacatgcctggctaatttttgtatatttagtagagacgaggtttcaccatgttggccaggctgatcttgaattcctgacctcaggttatccacctgcctcggcctcccaaagtgctaggattacaggcgtgagccaccacgcccagctgattatccatataattataacactcttctatttattttcagtcaccaataattccttttgagcaatatttaagcctagcatatttcttccttccctcctcctctactaaccagttctggtcgatatattattggattttactcttatactgtttgtttgtttgtttgtttgtttattttgagacagagtcttgctctgttgctgaggctggagtacagtggtgtgatctgagctcacggcaccctccacctcctagcttcgtgcgattctgatgcttcaaccttccgagtagctgggattacaggcatgcgccaccatgtcgggctaatttttgtgtttttagtaaaggcgaggtttcaccatgttggatgatcttgaactcctggcttcaagagatctatctgcctcagcctcccaaagtgctgggattacaagcataatccaccacacctgacctacttttgtatgttaaatgtgattatacttctctttgacttgtcagcttagctttagctgatacactctggtgcccaactattattgtatcagtgaacttccactttcttttccttttctctcaatttttgttgtatcattcctaccttgtgaggacatataatatttacattctgttgtcatcctcacatttcttagttccacagtttaaatgtatttgaaactcaaaacattcccattaatctcttggtcagctgaaattaatgatttaatagtttccttaaaaaagactcatggaacaatttccctaaatttttgccatgtcaaatatgtttatctgtagcctttacacagtaaaaacaatttggctagataatacaattctcagttcatatttttctttggaatattaaagtattgctatagagaaaaaaaaaaaaaaaa

SEQ ID NO: 20 - protein, 107 aa, Homo sapiens
MEQKLVEEILQAITMSTDTGVSLPSYEEDQGSKLIRKAKEAPFVPVGIAGFAAIVAYGLYKLKSRGNTKMSIHLIHMRVAAQGFVVGAMTVGMGYSMYREFWAKPKP

SEQ ID NO: 21 - DNA, 2805 bp, Homo sapiens
gattggctgggacggctgtgggtggggagaagccgggaggactgggtgcgcctgcagggatcggaagccggttggggtgtgagaggttttctcgctctagaacctcatagaaattctttctcagggagattcttcaagcaatcactatgtcaacagacacaggtgtttcccttccttcatatgaggaagatcagggatcaaaactcattcgaaaagctaaagaggcaccattcgtacccgttggaatagcgggttttgcagcaattgttgcatatggattatataaactgaagagcaggggaaatactaaaatgtccattcatctgatccacatgcgtgtggcagcccaaggctttgttgtaggagcaatgactgttggtatgggctattccatgtatcgggaattctgggcaaaacctaagccttagaagaagagatgctgtcttggtcttgttggaggagcttgctttagttagatgtcttattattaaagttacctattattgttggaaataaactaatttgtatgggtttagatggtaacatggcattttgaatattggcttcctttcttgcaggcttgatttgcttggtgaccgaattactagtgactagtttactaactaggtcattcaaggaagtcaagttaacttaaacatgtcacctaaatgcacttgatggtgttgaaatgtccaccttcttaaatttttaagatgaacttagttctaaagaagataacaggccaatcctgaaggtactccctgtttgctgcagaatgtcagatattttggatgttgcataagagtcctatttgccccagttaattcaacttttgtctgcctgttttgtggactggctggctctgttagaactctgtccaaaaagtgcatggaatataacttgtaaagcttcccacaattgacaatatatatgcatgtgtttaaaccaaatccagaaagcttaaacaatagagctgcataatagtatttattaaagaatcacaactgtaaacatgagaataatttaaggattctagtttagttttttgtaattgcaaattatatttttgctgctgatatattagaataatttttaaatgtcatcttgaaatagaaatatgtattttaagcactcacgcaaaggtaaatgaacacgttttaaatgtgtgtgttgctaattttttccataagaattgtaaacattgaactgaacaaattacctataatggatttggttaatgacttatgagcaagctggtttggccagacagtatacccaaacttttatataatatacagaaggctatcacacttgtgaaattctcttgtctaatctgaatttgcattccatggtgttaacatggtatatgtattgttattaaagtaagtgacccatgtcaaatgtcttttatttatttcatgaggaaaagctttctgtagaggaacaaatttgagaacaagtttcaggaaattgtcttttttgttgttgttctctaatcatgttctcctttctgtttcaacgattttaaaaatattttactttatggtatgttttattttttttccttttgtgggtaatttttgttctattgattatccatataaattttttttttttttttttgagacggagttattctctgtcatcttggctggcgtgcagtggcacgatcttggctcactgcaacttccatcccccaggttcaagtgattctcttgcctcagcctcctgagtagctgtgattacaggcatgcaccaacatgcctggctaatttttgtatatttagtagagacgaggtttcaccatgttggccaggctgatcttgaattcctgacctcaggttatccacctgcctcggcctcccaaagtgctaggattacaggcgtgagccaccacgcccagctgattatccatataattataacactcttctatttattttcagtcaccaataattccttttgagcaatatttaagcctagcatatttcttccttccctcctcctctactaaccagttctggtcgatatattattggattttactcttatactgtttgtttgtttgtttgtttgtttattttgagacagagtcttgctctgttgctgaggctggagtacagtggtgtgatctgagctcacggcaccctccacctcctagcttcgtgcgattctgatgcttcaaccttccgagtagctgggattacaggcatgcgccaccatgtcgggctaatttttgtgtttttagtaaaggcgaggtttcaccatgttggatgatcttgaactcctggcttcaagagatctatctgcctcagcctcccaaagtgctgggattacaagcataatccaccacacctgacctacttttgtatgttaaatgtgattatacttctctttgacttgtcagcttagctttagctgatacactctggtgcccaactattattgtatcagtgaacttccactttcttttccttttctctcaatttttgttgtatcattcctaccttgtgaggacatataatatttacattctgttgtcatcctcacatttcttagttccacagtttaaatgtatttgaaactcaaaacattcccattaatctcttggtcagctgaaattaatgatttaatagtttccttaaaaaagactcatggaacaatttccctaaatttttgccatgtcaaatatgtttatctgtagcctttacacagtaaaaacaatttggctagataatacaattctcagttcatatttttctttggaatattaaagtattgctatagagaaaaaaaaaaaaaaaa

SEQ ID NO: 22 - protein, 93 aa, Homo sapiens [sequence omitted]

SEQ ID NO: 23 - DNA, 1661 bp, Homo sapiens
aagtcgcggccaatgggcgacgcggccgcagatccgcccggccccgccctgccctgtgagttcctccggccgggctgcggggctccgctcagtccgggagcgcagctgggccgcggcgctccgacctccgctttcccaccgcccgcagctgaagcacatcccgcagcccggcgcggactccgatcgccgcagttgccctctggcgccatgtcgcagaacggagcgcccgggatgcaggaggagagcctgcagggctcctgggtagaactgcacttcagcaataatgggaacgggggcagcgttccagcctcggtttctatttataatggagacatggaaaaaatactgctggacgcacagcatgagtctggacggagtagctccaagagctctcactgtgacagcccacctcgctcgcagacaccacaagataccaacagagcttctgaaacagatacccatagcattggagagaaaaacagctcacagtctgaggaagatgatattgaaagaaggaaagaagttgaaagcatcttgaagaaaaactcagattggatatgggattggtcaagtcggccggaaaatattccccccaaggagttcctctttaaacacccgaagcgcacggccaccctcagcatgaggaacacgagcgtcatgaagaaagggggcatattctctgcagaatttctgaaagttttccttccatctctgctgctctctcatttgctggccatcggattggggatctatattggaaggcgtctgacaacctccaccagcaccttttgatgaagaactggagtctgacttggttcgttagtggattacttctgagcttgcaacatagctcactgaagagctgttagatcctggggtggccacgtcacttgtgtttatttgttctgtaaatgctgcgttcctaatttagtaaaataaaagaatagacactaaaatcatgttgatctataattacacctatgggatcaataagcatgtcagactgattaatgtctactgtgaaaatttggtagtaaattttcatttgatattagatataaatatctgaatataaataattttaatatactagtcatgatgtgtgttgtattttaaaaattatctgcaaccttaattcagctgaagtactttatatttcaaaagaatgaataacattgataataaaatcgctactttaaggggtttgtccaaaataaatattgtggccttatatatcacactattgtagaaagtattatttaatttaaatggatgcaggttgtctactaaagaaagattatatataactatgctaattgttcataatcaacagaaaccaagatagagctacaaactcagctgtacagttcgtacactaaactcttcttgcttttgcattataaggaattaagtctccgattattaggtgatcaccctggatgatcagttttctgctgaaggcacctactcagtatcttttcctctttatcactctgcattggtgaatttaatcctctcctttgtgttcaacttttgtgtgcttttaaaatcagctttattctaagcaaatctgtgtctactttaaaaaactggaaatggaaaaaaaaataaatctttgccaaatccttcagataaaaaaaaaaaaaaaaaaaaaaaaaaaa

SEQ ID NO: 24 - protein, 259 aa, Homo sapiens
MGDAAADPPGPALPCEFLRPGCGAPLSPGAQLGRGAPTSAFPPPAAEAHPAARRGLRSPQLPSGAMSQNGAPGMQEESLQGSWVELHFSNNGNGGSVPASVSIYNGDMEKILLDAQHESGRSSSKSSHCDSPPRSQTPQDTNRASETDTHSIGEKNSSQSEEDDIERRKEVESILKKNSDWIWDWSSRPENIPPKEFLFKHPKRTATLSMRNTSVMKKGGIFSAEFLKVFLPSLLLSHLLAIGLGIYIGRRLTTSTSTF

SEQ ID NO: 25 - DNA, 4403 bp, Homo sapiens
actgttgagttagcgcctcgccttccggggcggattgtctgtcgttgcagtagctgtaggaaggggaggccattttccgtttctgggaggagtgaggggcaacgggtcggagaaaaaggaaaaaagaagggctcagcgcctccccgccgggccgtggacagaggggcacagtttcggcaggcgggtgaggtcgctgagggcccgccggagatgttttccttgtcgagcacggtgcaaccccaggttacagttcctctgagtcatctcatcaatgccttccatacaccaaaaaacacttctgtttctctcagtggagtgtcagtttctcaaaaccagcatcgagatgtagttcctgagcatgaggctcccagcagtgagtgtatgttcagtgacttcctgacgaagcttaacattgtttcaattggcaaaggaaaaatattcgaagggtacagatccatgttcatggagccagcaaaaaggatgaagaagagcttggacacaaccgataactggcacatccgtccagaacccttctccctctcaatccctccttcacttaacttaagggaccttggattatctgaactaaaaattggacagattgatcagctggtagaaaatctacttcctggattttgtaaaggcaaaaacatttcttcccattggcatacatcccatgtctctgcacaatccttctttgaaaataaatatggtaacttagatatatttagtacattacgttcctcttgcttgtatcgacatcattcaagagctcttcaaagcatttgttcagatcttcagtactggccagttttcatacagtctcggggttttaaaactttgaaatcaaggacacgacgtctccagtctacctccgagagattagctgaaacacagaatatagcgccatcattcgtgaaggggtttcttttgcgggacagaggatcagatgttgagagtttggacaaactcatgaaaaccaaaaatatacctgaagctcaccaagatgcatttaaaactggttttgcggaaggttttctgaaagctcaagcactcacacaaaaaaccaatgattccctaaggcgaacccgtctgattctcttcgttctgctgctattcggcatttatggacttctaaaaaacccatttttatctgtccgcttccggacaacaacagggcttgattctgcagtagatcctgtccagatgaaaaatgtcacctttgaacatgttaaaggggtggaggaagctaaacaagaattacaggaagttgttgaattcttgaaaaatccacaaaaatttactattcttggaggtaaacttccaaaaggaattcttttagttggacccccagggactggaaagacacttcttgcccgagctgtggcgggagaagctgatgttcctttttattatgcttctggatccgaatttgatgagatgtttgtgggtgtgggagccagccgtatcagaaatctttttagggaagcaaaggcgaatgctccttgtgttatatttattgatgaattagattctgttggtgggaagagaattgaatctccaatgcatccatattcaaggcagaccataaatcaacttcttgctgaaatggatggttttaaacccaatgaaggagttatcataataggagccacaaacttcccagaggcattagataatgccttaatacgtcctggtcgttttgacatgcaagttacagttccaaggccagatgtaaaaggtcgaacagaaattttgaaatggtatctcaataaaataaagtttgatcaatccgttgatccagaaattatagctcgaggtactgttggcttttccggagcagagttggagaatcttgtgaaccaggctgcattaaaagcagctgttgatggaaaagaaatggttaccatgaaggagctggagttttccaaagacaaaattctaatggggcctgaaagaagaagtgtggaaattgataacaaaaacaaaaccatcacagcatatcatgaatctggtcatgccattattgcatattacacaaaagatgcaatgcctatcaacaaagctacaatcatgccacgggggccaacacttggacatgtgtccctgttacctgagaatgacagatggaatgaaactagagcccagctgcttgcacaaatggatgttagtatgggaggaagagtggcagaggagcttatatttggaaccgaccatattacaacaggtgcttccagtgattttgataatgccactaaaatagcaaagcggatggttaccaaatttggaatgagtgaaaagcttggagttatgacctacagtgatacagggaaactaagtccagaaacccaatctgccatcgaacaagaaataagaatccttctaagggactcatatgaacgagcaaaacatatcttgaaaactcatgcaaaggagcataagaatctcgcagaagctttattgacctatgagactttggatgccaaagagattcaaattgttcttgaggggaaaaagttggaagtgagatgataactctcttgatatggatgcttgctggttttattgcaagaatacaagtagcattgcagtagtctacttttacaacgctttcccctcattcttgatgtggtgtaattgaagggtgtgaaatgctttgtcaatcatttgtcacatttatccagtttgggttattctcattatgacacctattgcaaattagcatcccatggcaaatatattttgaaaaaataaagaactatcaggattgaaaacagctcttttgaggaatgtcaattagttattaagttgaaagtaattaatgattttatgtttggttactctactagatttgataaaaattgtgcctttagccttctatatacatcagtggaaacttaagatgcagtaattatgttccagattgaccatgaataaaatattttttaatctaaatgtagagaagttgggattaaaagcagtctcggaaacacagagccaggaatatagccttttggcatggtgccatggctcacatctgtaatcccagcacttttggaggctgaggcgggtggattgcttgaggccaggagttcgagaccagcctggccaacgtggtgaaacgctgtctctactaaaatacaaaaaaatagggctgggcgcggttgctcacgcctgtaatcccagcacttttcagaggccaaggcgggcaaatcacctgaggtcaagagtttgagaccagcctggccaacatggtgaaaccccatctctactaaacatgcaaaaattacctgggcatggtggcaggtgcttataatcccagctactctgggggccaaggcaggagaattgcttgagcctgggagatggaggttgcagtgagctgagatcatgccactgcactccagcctgggcaacagagcaagactctgcctcaaaaaaaaattaaaataaatttaaatacaaaaaaaaatagccaggtgtggggtgcatgcctggaatcccagctacttgagaggctgaggcacgagaattgcttgaacccaggaggtggaggttgcagtgagccaagatcacaggagccactgcactccagcctgggtgacagagtgagactctgtctcaaaaaaaaattaaataaattattataacctttcagaaatgctgtgtgcattttcatgttcttttttttagcattactgtcactctccctaatgaaatgtacttcagagaagcagtattttgttaaataaatacataacctcattctgaataatgtccctcattttgactataactgtgcttggtttcaaaagcaaaattaaacaaaaatctcagtcccctccgaagtgaactttgtgttaccctgcgtcagaaatgccaagttgtgtttacttttcattcagattttgtgaatatgaacatgctgttataggatctacagatgaatatttaactcaatagaaaaattattttagaacacattgtattggtattacaaccagattatattcttgacgttgacttcattaaaattatctacaatttcctaataatttaagctgtatatggtcttcattgaaaaaagatagatattgttacaggaagcttgttacattatattcttgaccttttggttgataatcttaaatcttaatgtaatttcaaactggcagaaatgttgccagcataatacatggatgtctcatataccctgcatccagatttaccagttgttatcattctgcccgttttttattgccccaaacctgttctgtctccctctctgtatgtacatacatacacgtataaaatattgataaagtcttatctgtcttaaatttttttacatatttgttgaggtataatttacatatgataaaattcattttaaatgtaaaaaa

SEQ ID NO: 26 - protein, 773 aa, Homo sapiens
MFSLSSTVQPQVTVPLSHLINAFHTPKNTSVSLSGVSVSQNQHRDVVPEHEAPSSECMFSDFLTKLNIVSIGKGKIFEGYRSMFMEPAKRMKKSLDTTDNWHIRPEPFSLSIPPSLNLRDLGLSELKIGQIDQLVENLLPGFCKGKNISSHWHTSHVSAQSFFENKYGNLDIFSTLRSSCLYRHHSRALQSICSDLQYWPVFIQSRGFKTLKSRTRRLQSTSERLAETQNIAPSFVKGFLLRDRGSDVESLDKLMKTKNIPEAHQDAFKTGFAEGFLKAQALTQKTNDSLRRTRLILFVLLLFGIYGLLKNPFLSVRFRTTTGLDSAVDPVQMKNVTFEHVKGVEEAKQELQEVVEFLKNPQKFTILGGKLPKGILLVGPPGTGKTLLARAVAGEADVPFYYASGSEFDEMFVGVGASRIRNLFREAKANAPCVIFIDELDSVGGKRIESPMHPYSRQTINQLLAEMDGFKPNEGVIIIGATNFPEALDNALIRPGRFDMQVTVPRPDVKGRTEILKWYLNKIKFDQSVDPEIIARGTVGFSGAELENLVNQAALKAAVDGKEMVTMKELEFSKDKILMGPERRSVEIDNKNKTITAYHESGHAIIAYYTKDAMPINKATIMPRGPTLGHVSLLPENDRWNETRAQLLAQMDVSMGGRVAEELIFGTDHITTGASSDFDNATKIAKRMVTKFGMSEKLGVMTYSDTGKLSPETQSAIEQEIRILLRDSYERAKHILKTHAKEHKNLAEALLTYETLDAKEIQIVLEGKKLEVR

SEQ ID NO: 27 - DNA, 4232 bp, Homo sapiens
actgttgagttagcgcctcgccttccggggcggattgtctgtcgttgcagtagctgtaggaaggggaggccattttccgtttctgggaggagtgaggggcaacgggtcggagaaaaaggaaaaaagaagggctcagcgcctccccgccgggccgtggacagaggggcacagtttcggcaggcgggtgaggtcgctgagggcccgccggagatgttttccttgtcgagcacggtgcaaccccaggttacagttcctctgagtcatctcatcaatgccttccatacaccaaaaaacacttctgtttctctcagtggagtgtcagtttctcaaaaccagcatcgagatgtagttcctgagcatgaggctcccagcagtgagccttcacttaacttaagggaccttggattatctgaactaaaaattggacagattgatcagctggtagaaaatctacttcctggattttgtaaaggcaaaaacatttcttcccattggcatacatcccatgtctctgcacaatccttctttgaaaataaatatggtaacttagatatatttagtacattacgttcctcttgcttgtatcgacatcattcaagagctcttcaaagcatttgttcagatcttcagtactggccagttttcatacagtctcggggttttaaaactttgaaatcaaggacacgacgtctccagtctacctccgagagattagctgaaacacagaatatagcgccatcattcgtgaaggggtttcttttgcgggacagaggatcagatgttgagagtttggacaaactcatgaaaaccaaaaatatacctgaagctcaccaagatgcatttaaaactggttttgcggaaggttttctgaaagctcaagcactcacacaaaaaaccaatgattccctaaggcgaacccgtctgattctcttcgttctgctgctattcggcatttatggacttctaaaaaacccatttttatctgtccgcttccggacaacaacagggcttgattctgcagtagatcctgtccagatgaaaaatgtcacctttgaacatgttaaaggggtggaggaagctaaacaagaattacaggaagttgttgaattcttgaaaaatccacaaaaatttactattcttggaggtaaacttccaaaaggaattcttttagttggacccccagggactggaaagacacttcttgcccgagctgtggcgggagaagctgatgttcctttttattatgcttctggatccgaatttgatgagatgtttgtgggtgtgggagccagccgtatcagaaatctttttagggaagcaaaggcgaatgctccttgtgttatatttattgatgaattagattctgttggtgggaagagaattgaatctccaatgcatccatattcaaggcagaccataaatcaacttcttgctgaaatggatggttttaaacccaatgaaggagttatcataataggagccacaaacttcccagaggcattagataatgccttaatacgtcctggtcgttttgacatgcaagttacagttccaaggccagatgtaaaaggtcgaacagaaattttgaaatggtatctcaataaaataaagtttgatcaatccgttgatccagaaattatagctcgaggtactgttggcttttccggagcagagttggagaatcttgtgaaccaggctgcattaaaagcagctgttgatggaaaagaaatggttaccatgaaggagctggagttttccaaagacaaaattctaatggggcctgaaagaagaagtgtggaaattgataacaaaaacaaaaccatcacagcatatcatgaatctggtcatgccattattgcatattacacaaaagatgcaatgcctatcaacaaagctacaatcatgccacgggggccaacacttggacatgtgtccctgttacctgagaatgacagatggaatgaaactagagcccagctgcttgcacaaatggatgttagtatgggaggaagagtggcagaggagcttatatttggaaccgaccatattacaacaggtgcttccagtgattttgataatgccactaaaatagcaaagcggatggttaccaaatttggaatgagtgaaaagcttggagttatgacctacagtgatacagggaaactaagtccagaaacccaatctgccatcgaacaagaaataagaatccttctaagggactcatatgaacgagcaaaacatatcttgaaaactcatgcaaaggagcataagaatctcgcagaagctttattgacctatgagactttggatgccaaagagattcaaattgttcttgaggggaaaaagttggaagtgagatgataactctcttgatatggatgcttgctggttttattgcaagaatacaagtagcattgcagtagtctacttttacaacgctttcccctcattcttgatgtggtgtaattgaagggtgtgaaatgctttgtcaatcatttgtcacatttatccagtttgggttattctcattatgacacctattgcaaattagcatcccatggcaaatatattttgaaaaaataaagaactatcaggattgaaaacagctcttttgaggaatgtcaattagttattaagttgaaagtaattaatgattttatgtttggttactctactagatttgataaaaattgtgcctttagccttctatatacatcagtggaaacttaagatgcagtaattatgttccagattgaccatgaataaaatattttttaatctaaatgtagagaagttgggattaaaagcagtctcggaaacacagagccaggaatatagccttttggcatggtgccatggctcacatctgtaatcccagcacttttggaggctgaggcgggtggattgcttgaggccaggagttcgagaccagcctggccaacgtggtgaaacgctgtctctactaaaatacaaaaaaatagggctgggcgcggttgctcacgcctgtaatcccagcacttttcagaggccaaggcgggcaaatcacctgaggtcaagagtttgagaccagcctggccaacatggtgaaaccccatctctactaaacatgcaaaaattacctgggcatggtggcaggtgcttataatcccagctactctgggggccaaggcaggagaattgcttgagcctgggagatggaggttgcagtgagctgagatcatgccactgcactccagcctgggcaacagagcaagactctgcctcaaaaaaaaattaaaataaatttaaatacaaaaaaaaatagccaggtgtggggtgcatgcctggaatcccagctacttgagaggctgaggcacgagaattgcttgaacccaggaggtggaggttgcagtgagccaagatcacaggagccactgcactccagcctgggtgacagagtgagactctgtctcaaaaaaaaattaaataaattattataacctttcagaaatgctgtgtgcattttcatgttcttttttttagcattactgtcactctccctaatgaaatgtacttcagagaagcagtattttgttaaataaatacataacctcattctgaataatgtccctcattttgactataactgtgcttggtttcaaaagcaaaattaaacaaaaatctcagtcccctccgaagtgaactttgtgttaccctgcgtcagaaatgccaagttgtgtttacttttcattcagattttgtgaatatgaacatgctgttataggatctacagatgaatatttaactcaatagaaaaattattttagaacacattgtattggtattacaaccagattatattcttgacgttgacttcattaaaattatctacaatttcctaataatttaagctgtatatggtcttcattgaaaaaagatagatattgttacaggaagcttgttacattatattcttgaccttttggttgataatcttaaatcttaatgtaatttcaaactggcagaaatgttgccagcataatacatggatgtctcatataccctgcatccagatttaccagttgttatcattctgcccgttttttattgccccaaacctgttctgtctccctctctgtatgtacatacatacacgtataaaatattgataaagtcttatctgtcttaaatttttttacatatttgttgaggtataatttacatatgataaaattcattttaaatgtaaaaaa

SEQ ID NO: 28 - protein, 716 aa, Homo sapiens
MFSLSSTVQPQVTVPLSHLINAFHTPKNTSVSLSGVSVSQNQHRDVVPEHEAPSSEPSLNLRDLGLSELKIGQIDQLVENLLPGFCKGKNISSHWHTSHVSAQSFFENKYGNLDIFSTLRSSCLYRHHSRALQSICSDLQYWPVFIQSRGFKTLKSRTRRLQSTSERLAETQNIAPSFVKGFLLRDRGSDVESLDKLMKTKNIPEAHQDAFKTGFAEGFLKAQALTQKTNDSLRRTRLILFVLLLFGIYGLLKNPFLSVRFRTTTGLDSAVDPVQMKNVTFEHVKGVEEAKQELQEVVEFLKNPQKFTILGGKLPKGILLVGPPGTGKTLLARAVAGEADVPFYYASGSEFDEMFVGVGASRIRNLFREAKANAPCVIFIDELDSVGGKRIESPMHPYSRQTINQLLAEMDGFKPNEGVIIIGATNFPEALDNALIRPGRFDMQVTVPRPDVKGRTEILKWYLNKIKFDQSVDPEIIARGTVGFSGAELENLVNQAALKAAVDGKEMVTMKELEFSKDKILMGPERRSVEIDNKNKTITAYHESGHAIIAYYTKDAMPINKATIMPRGPTLGHVSLLPENDRWNETRAQLLAQMDVSMGGRVAEELIFGTDHITTGASSDFDNATKIAKRMVTKFGMSEKLGVMTYSDTGKLSPETQSAIEQEIRILLRDSYERAKHILKTHAKEHKNLAEALLTYETLDAKEIQIVLEGKKLEVR

SEQ ID NO: 29 - DNA, 4133 bp, Homo sapiens
actgttgagttagcgcctcgccttccggggcggattgtctgtcgttgcagtagctgtaggaaggggaggccattttccgtttctgggaggagtgaggggcaacgggtcggagaaaaaggaaaaaagaagggctcagcgcctccccgccgggccgtggacagaggggcacagtttcggcaggcgggtgaggtcgctgagggcccgccggagatgttttccttgtcgagcacggtgcaaccccaggttacagttcctctgagtcatctcatcaatgccttccatacaccaaaaaacacttctgtttctctcagtggagtgtcagtttctcaaaaccagcatcgagatgtagttcctgagcatgaggctcccagcagtgagccttcacttaacttaagggaccttggattatctgaactaaaaattggacagattgatcagctggtagaaaatctacttcctggattttgtaaaggcaaaaacatttcttcccattggcatacatcccatgtctctgcacaatccttctttgaaaataaatatgttttcatacagtctcggggttttaaaactttgaaatcaaggacacgacgtctccagtctacctccgagagattagctgaaacacagaatatagcgccatcattcgtgaaggggtttcttttgcgggacagaggatcagatgttgagagtttggacaaactcatgaaaaccaaaaatatacctgaagctcaccaagatgcatttaaaactggttttgcggaaggttttctgaaagctcaagcactcacacaaaaaaccaatgattccctaaggcgaacccgtctgattctcttcgttctgctgctattcggcatttatggacttctaaaaaacccatttttatctgtccgcttccggacaacaacagggcttgattctgcagtagatcctgtccagatgaaaaatgtcacctttgaacatgttaaaggggtggaggaagctaaacaagaattacaggaagttgttgaattcttgaaaaatccacaaaaatttactattcttggaggtaaacttccaaaaggaattcttttagttggacccccagggactggaaagacacttcttgcccgagctgtggcgggagaagctgatgttcctttttattatgcttctggatccgaatttgatgagatgtttgtgggtgtgggagccagccgtatcagaaatctttttagggaagcaaaggcgaatgctccttgtgttatatttattgatgaattagattctgttggtgggaagagaattgaatctccaatgcatccatattcaaggcagaccataaatcaacttcttgctgaaatggatggttttaaacccaatgaaggagttatcataataggagccacaaacttcccagaggcattagataatgccttaatacgtcctggtcgttttgacatgcaagttacagttccaaggccagatgtaaaaggtcgaacagaaattttgaaatggtatctcaataaaataaagtttgatcaatccgttgatccagaaattatagctcgaggtactgttggcttttccggagcagagttggagaatcttgtgaaccaggctgcattaaaagcagctgttgatggaaaagaaatggttaccatgaaggagctggagttttccaaagacaaaattctaatggggcctgaaagaagaagtgtggaaattgataacaaaaacaaaaccatcacagcatatcatgaatctggtcatgccattattgcatattacacaaaagatgcaatgcctatcaacaaagctacaatcatgccacgggggccaacacttggacatgtgtccctgttacctgagaatgacagatggaatgaaactagagcccagctgcttgcacaaatggatgttagtatgggaggaagagtggcagaggagcttatatttggaaccgaccatattacaacaggtgcttccagtgattttgataatgccactaaaatagcaaagcggatggttaccaaatttggaatgagtgaaaagcttggagttatgacctacagtgatacagggaaactaagtccagaaacccaatctgccatcgaacaagaaataagaatccttctaagggactcatatgaacgagcaaaacatatcttgaaaactcatgcaaaggagcataagaatctcgcagaagctttattgacctatgagactttggatgccaaagagattcaaattgttcttgaggggaaaaagttggaagtgagatgataactctcttgatatggatgcttgctggttttattgcaagaatacaagtagcattgcagtagtctacttttacaacgctttcccctcattcttgatgtggtgtaattgaagggtgtgaaatgctttgtcaatcatttgtcacatttatccagtttgggttattctcattatgacacctattgcaaattagcatcccatggcaaatatattttgaaaaaataaagaactatcaggattgaaaacagctcttttgaggaatgtcaattagttattaagttgaaagtaattaatgattttatgtttggttactctactagatttgataaaaattgtgcctttagccttctatatacatcagtggaaacttaagatgcagtaattatgttccagattgaccatgaataaaatattttttaatctaaatgtagagaagttgggattaaaagcagtctcggaaacacagagccaggaatatagccttttggcatggtgccatggctcacatctgtaatcccagcacttttggaggctgaggcgggtggattgcttgaggccaggagttcgagaccagcctggccaacgtggtgaaacgctgtctctactaaaatacaaaaaaatagggctgggcgcggttgctcacgcctgtaatcccagcacttttcagaggccaaggcgggcaaatcacctgaggtcaagagtttgagaccagcctggccaacatggtgaaaccccatctctactaaacatgcaaaaattacctgggcatggtggcaggtgcttataatcccagctactctgggggccaaggcaggagaattgcttgagcctgggagatggaggttgcagtgagctgagatcatgccactgcactccagcctgggcaacagagcaagactctgcctcaaaaaaaaattaaaataaatttaaatacaaaaaaaaatagccaggtgtggggtgcatgcctggaatcccagctacttgagaggctgaggcacgagaattgcttgaacccaggaggtggaggttgcagtgagccaagatcacaggagccactgcactccagcctgggtgacagagtgagactctgtctcaaaaaaaaattaaataaattattataacctttcagaaatgctgtgtgcattttcatgttcttttttttagcattactgtcactctccctaatgaaatgtacttcagagaagcagtattttgttaaataaatacataacctcattctgaataatgtccctcattttgactataactgtgcttggtttcaaaagcaaaattaaacaaaaatctcagtcccctccgaagtgaactttgtgttaccctgcgtcagaaatgccaagttgtgtttacttttcattcagattttgtgaatatgaacatgctgttataggatctacagatgaatatttaactcaatagaaaaattattttagaacacattgtattggtattacaaccagattatattcttgacgttgacttcattaaaattatctacaatttcctaataatttaagctgtatatggtcttcattgaaaaaagatagatattgttacaggaagcttgttacattatattcttgaccttttggttgataatcttaaatcttaatgtaatttcaaactggcagaaatgttgccagcataatacatggatgtctcatataccctgcatccagatttaccagttgttatcattctgcccgttttttattgccccaaacctgttctgtctccctctctgtatgtacatacatacacgtataaaatattgataaagtcttatctgtcttaaatttttttacatatttgttgaggtataatttacatatgataaaattcattttaaatgtaaaaaa

SEQ ID NO: 30 - protein, 683 aa, Homo sapiens
MFSLSSTVQPQVTVPLSHLINAFHTPKNTSVSLSGVSVSQNQHRDVVPEHEAPSSEPSLNLRDLGLSELKIGQIDQLVENLLPGFCKGKNISSHWHTSHVSAQSFFENKYVFIQSRGFKTLKSRTRRLQSTSERLAETQNIAPSFVKGFLLRDRGSDVESLDKLMKTKNIPEAHQDAFKTGFAEGFLKAQALTQKTNDSLRRTRLILFVLLLFGIYGLLKNPFLSVRFRTTTGLDSAVDPVQMKNVTFEHVKGVEEAKQELQEVVEFLKNPQKFTILGGKLPKGILLVGPPGTGKTLLARAVAGEADVPFYYASGSEFDEMFVGVGASRIRNLFREAKANAPCVIFIDELDSVGGKRIESPMHPYSRQTINQLLAEMDGFKPNEGVIIIGATNFPEALDNALIRPGRFDMQVTVPRPDVKGRTEILKWYLNKIKFDQSVDPEIIARGTVGFSGAELENLVNQAALKAAVDGKEMVTMKELEFSKDKILMGPERRSVEIDNKNKTITAYHESGHAIIAYYTKDAMPINKATIMPRGPTLGHVSLLPENDRWNETRAQLLAQMDVSMGGRVAEELIFGTDHITTGASSDFDNATKIAKRMVTKFGMSEKLGVMTYSDTGKLSPETQSAIEQEIRILLRDSYERAKHILKTHAKEHKNLAEALLTYETLDAKEIQIVLEGKKLEVR

SEQ ID NO: 31 - DNA, 1919 bp, Homo sapiens
atgtggaggtcagagtggaagcaggtgagaatggagggggcggcaaaggctcgtttctgggcatctctgcagtcctcctctgctccatgatgtgcactttgggcgaggagagtgcgtgcgtgtgagagggtccagcagaaggaaacatggctgccaaagtgtttgagtccattggcaagtttggcctggccttagctgttgcaggaggcgtggtgaactctgccttatataatgtggatgctgggcacagagctgtcatctttgaccgattccgtggagtgcaggacattgtggtaggggaagggactcattttctcatcccgtgggtacagaaaccaattatctttgactgccgttctcgaccacgtaatgtgccagtcatcactggtagcaaagatttacagaatgtcaacatcacactgcgcatcctcttccggcctgtcgccagccagcttcctcgcatcttcaccagcatcggagaggactatgatgagcgtgtgctgccgtccatcacaactgagatcctcaagtcagtggtggctcgctttgatgctggagaactaatcacccagagagagctggtctccaggcaggtgagcgacgaccttacagagcgagccgccacctttgggctcatcctggatgacgtgtccttgacacatctgaccttcgggaaggagttcacagaagcggtggaagccaaacaggtggctcagcaggaagcagagagggccagatttgtggtggaaaaggctgagcaacagaaaaaggcggccatcatctctgctgagggcgactccaaggcagctgagctgattgccaactcactggccactgcaggggatggcctgatcgagctgcgcaagctggaagctgcagaggacatcgcgtaccagctctcacgctctcggaacatcacctacctgccagcggggcagtccgtgctcctccagctgccccagtgagggcccaccctgcctgcacctccgcgggctgactgggccacagccccgatgattcttaacacagccttccttctgctcccaccccagaaatcactgtgaaatttcatgattggcttaaagtgaaggaaataaaggtaaaatcacttcagatctctaattagtctatcaaatgaaactctttcattcttctcacatccatctacttttttatccacctccctaccaaaaattgccaagtgcctatgcaaaccagctttaggtcccaattcggggcctgctggagttccggcctgggcaccagcatttggcagcacgcaggcggggcagtatgtgatggactggggagcacaggtgtctgcctagatccacgtgtggcctccgtcctgtcactgatggaaggtttgcggatgagggcatgtgcggctgaactgagaaggcaggcctccgtcttcccagcggttcctgtgcagatgctgctgaagagaggtgccggggaggggcagagaggaagtggtctgtctgttaccataagtctgattctctttaactgtgtgaccagcggaaacaggtgtgtgtgaactgggcacagattgaagaatctgcccctgttgaggtgggtgggcctgactgttgccccccagggtcctaaaacttggatggacttgtatagtgagagaggaggcctggaccgagatgtgagtcctgttgaagacttcctctctaccccccaccttggtccctctcagatacccagtggaattccaacttgaaggattgcatcctgctggggctgaacatgcctgccaaagacgtgtccgacctacgttcctggccccctcgttcagagactgcccttctcacgggctctatgcctgcactgggaaggaaacaaatgtgtataaactgctgtcaataaatgacacccagaccttccggctcagccaaaaaaaaaaa

SEQ ID NO: 32 - protein, 272 aa, Homo sapiens
MAAKVFESIGKFGLALAVAGGVVNSALYNVDAGHRAVIFDRFRGVQDIVVGEGTHFLIPWVQKPIIFDCRSRPRNVPVITGSKDLQNVNITLRILFRPVASQLPRIFTSIGEDYDERVLPSITTEILKSVVARFDAGELITQRELVSRQVSDDLTERAATFGLILDDVSLTHLTFGKEFTEAVEAKQVAQQEAERARFVVEKAEQQKKAAIISAEGDSKAAELIANSLATAGDGLIELRKLEAAEDIAYQLSRSRNITYLPAGQSVLLQLPQ

SEQ ID NO: 33 - DNA, 1520 bp, Homo sapiens
gggcggggcagaggagctcatgcgcagtatgtgtggttggggaattcatgtggaggtcagagtggaagcaggtgtgagagggtccagcagaaggaaacatggctgccaaagtgtttgagtccattggcaagtttggcctggccttagctgttgcaggaggcgtggtgaactctgccttatataatgtggatgctgggcacagagctgtcatctttgaccgattccgtggagtgcaggacattgtggtaggggaagggactcattttctcatcccgtgggtacagaaaccaattatctttgactgccgttctcgaccacgtaatgtgccagtcatcactggtagcaaagatttacagaatgtcaacatcacactgcgcatcctcttccggcctgtcgccagccagcttcctcgcatcttcaccagcatcggagaggactatgatgagcgtgtgctgccgtccatcacaactgagatcctcaagtcagtggtggctcgctttgatgctggagaactaatcacctacctgccagcggggcagtccgtgctcctccagctgccccagtgagggcccaccctgcctgcacctccgcgggctgactgggccacagccccgatgattcttaacacagccttccttctgctcccaccccagaaatcactgtgaaatttcatgattggcttaaagtgaaggaaataaaggtaaaatcacttcagatctctaattagtctatcaaatgaaactctttcattcttctcacatccatctacttttttatccacctccctaccaaaaattgccaagtgcctatgcaaaccagctttaggtcccaattcggggcctgctggagttccggcctgggcaccagcatttggcagcacgcaggcggggcagtatgtgatggactggggagcacaggtgtctgcctagatccacgtgtggcctccgtcctgtcactgatggaaggtttgcggatgagggcatgtgcggctgaactgagaaggcaggcctccgtcttcccagcggttcctgtgcagatgctgctgaagagaggtgccggggaggggcagagaggaagtggtctgtctgttaccataagtctgattctctttaactgtgtgaccagcggaaacaggtgtgtgtgaactgggcacagattgaagaatctgcccctgttgaggtgggtgggcctgactgttgccccccagggtcctaaaacttggatggacttgtatagtgagagaggaggcctggaccgagatgtgagtcctgttgaagacttcctctctaccccccaccttggtccctctcagatacccagtggaattccaacttgaaggattgcatcctgctggggctgaacatgcctgccaaagacgtgtccgacctacgttcctggccccctcgttcagagactgcccttctcacgggctctatgcctgcactgggaaggaaacaaatgtgtataaactgctgtcaataaatgacacccagaccttccggctcagccaaaaaaaaaaa

SEQ ID NO: 34 - protein, 155 aa, Homo sapiens
MAAKVFESIGKFGLALAVAGGVVNSALYNVDAGHRAVIFDRFRGVQDIVVGEGTHFLIPWVQKPIIFDCRSRPRNVPVITGSKDLQNVNITLRILFRPVASQLPRIFTSIGEDYDERVLPSITTEILKSVVARFDAGELITYLPAGQSVLLQLPQ

SEQ ID NO: 35 - DNA, 1457 bp, Homo sapiens
tccgtatgcgcgattcctgtgcgcgaagttcgggtccgtagtgggctaagggggagggtttcaaagggagcgcacttccgctgccctttctttcgccagccttacgggcccgaaccctcgtgtgaagggtgcagtacctaagccggagcggggtagaggcgggccggcacccccttctgacctccagtgccgccggcctcaagatcagacatggcccagaacttgaaggacttggcgggacggctgcccgccgggccccggggcatgggcacggccctgaagctgttgctgggggccggcgccgtggcctacggtgtgcgcgaatctgtgttcaccgtggaaggcgggcacagagccatcttcttcaatcggatcggtggagtgcagcaggacactatcctggccgagggccttcacttcaggatcccttggttccagtaccccattatctatgacattcgggccagacctcgaaaaatctcctcccctacaggctccaaagacctacagatggtgaatatctccctgcgagtgttgtctcgacccaatgctcaggagcttcctagcatgtaccagcgcctagggctggactacgaggaacgagtgttgccgtccattgtcaacgaggtgctcaagagtgtggtggccaagttcaatgcctcacagctgatcacccagcgggcccaggtatccctgttgatccgccgggagctgacagagagggccaaggacttcagcctcatcctggatgatgtggccatcacagagctgagctttagccgagagtacacagctgctgtagaagccaaacaagtggcccagcaggaggcccagcgggcccaattcttggtagaaaaagcaaagcaggaacagcggcagaaaattgtgcaggccgagggtgaggccgaggctgccaagatgcttggagaagcactgagcaagaaccctggctacatcaaacttcgcaagattcgagcagcccagaatatctccaagacgatcgccacatcacagaatcgtatctatctcacagctgacaaccttgtgctgaacctacaggatgaaagtttcaccaggggaagtgacagcctcatcaagggtaagaaatgagcctagtcaccaagaactccacccccagaggaagtggatctgcttctccagtttttgaggagccagccaggggtccagcacagccctaccccgccccagtatcatgcgatggtcccccacaccggttccctgaacccctcttggattaaggaagactgaagactagccccttttctggggaattactttcctcctccctgtgttaactggggctgttggggacagtgcgtgatttctcagtgatttcctacagtgttgttccctccctcaaggctgggaggagataaacaccaacccaggaattctcaataaatttttattacttaacctgaaaaaaaaaaaaaaaa

SEQ ID NO: 36 - protein, 299 aa, Homo sapiens
MAQNLKDLAGRLPAGPRGMGTALKLLLGAGAVAYGVRESVFTVEGGHRAIFFNRIGGVQQDTILAEGLHFRIPWFQYPIIYDIRARPRKISSPTGSKDLQMVNISLRVLSRPNAQELPSMYQRLGLDYEERVLPSIVNEVLKSVVAKFNASQLITQRAQVSLLIRRELTERAKDFSLILDDVAITELSFSREYTAAVEAKQVAQQEAQRAQFLVEKAKQEQRQKIVQAEGEAEAAKMLGEALSKNPGYIKLRKIRAAQNISKTIATSQNRIYLTADNLVLNLQDESFTRGSDSLIKGKK

SEQ ID NO: 37 - DNA, 1343 bp, Homo sapiens
tccgtatgcgcgattcctgtgcgcgaagttcgggtccgtagtgggctaagggggagggtttcaaagggagcgcacttccgctgccctttctttcgccagccttacgggcccgaaccctcgtgtgaagggtgcagtacctaagccggagcggggtagaggcgggccggcacccccttctgacctccagtgccgccggcctcaagatcagacatggcccagaacttgaaggacttggcgggacggctgcccgccgggccccggggcatgggcacggccctgaagctgttgctgggggccggcgccgtggcctacggtgtgcgcgaatctgtgttcaccgtggaaggcgggcacagagccatcttcttcaatcggatcggtggagtgcagcaggacactatcctggccgagggccttcacttcaggatcccttggttccagtaccccattatctatgacattcgggccagacctcgaaaaatctcctcccctacaggctccaaagacctacagatggtgaatatctccctgcgagtgttgtctcgacccaatgctcaggagcttcctagcatgtaccagcgcctagggctggactacgaggaacgagtgttgccgtccattgtcaacgaggtgctcaagagtgtggtggccaagttcaatgcctcacagctgatcacccagcgggcccaggtatccctgttgatccgccgggagctgacagagagggccaaggacttcagcctcatcctggatgatgtggccatcacagagctgagctttagccgagagtacacagctgctgtagaagccaaacaagtggcactgagcaagaaccctggctacatcaaacttcgcaagattcgagcagcccagaatatctccaagacgatcgccacatcacagaatcgtatctatctcacagctgacaaccttgtgctgaacctacaggatgaaagtttcaccaggggaagtgacagcctcatcaagggtaagaaatgagcctagtcaccaagaactccacccccagaggaagtggatctgcttctccagtttttgaggagccagccaggggtccagcacagccctaccccgccccagtatcatgcgatggtcccccacaccggttccctgaacccctcttggattaaggaagactgaagactagccccttttctggggaattactttcctcctccctgtgttaactggggctgttggggacagtgcgtgatttctcagtgatttcctacagtgttgttccctccctcaaggctgggaggagataaacaccaacccaggaattctcaataaatttttattacttaacctgaaaaaaaaaaaaaaaa

SEQ ID NO: 38 - protein, 261 aa, Homo sapiens
MAQNLKDLAGRLPAGPRGMGTALKLLLGAGAVAYGVRESVFTVEGGHRAIFFNRIGGVQQDTILAEGLHFRIPWFQYPIIYDIRARPRKISSPTGSKDLQMVNISLRVLSRPNAQELPSMYQRLGLDYEERVLPSIVNEVLKSVVAKFNASQLITQRAQVSLLIRRELTERAKDFSLILDDVAITELSFSREYTAAVEAKQVALSKNPGYIKLRKIRAAQNISKTIATSQNRIYLTADNLVLNLQDESFTRGSDSLIKGKK

SEQ ID NO: 39 - DNA, 1773 bp, Homo sapiens
aatgagcgaaggcatcgcgagccagggggcgcggagaaggcggggaatcatggccgcccccagtgttccgcgtccgggggtttgtgggagttgccttgacctgcagctccgccaccgcggacccgccttctgccctcagcagcagacgctctgtcccgcccgggcagctctgcgaggcagcggctggagagggaaccatggggactgtgcacgcccggagtttggagcctcttccatcaagtggacctgattttggaggattaggagaagaagctgaatttgttgaagttgagcctgaagctaaacaggaaattcttgaaaacaaagatgtggttgttcaacatgttcattttgatggacttggaaggactaaagatgatatcatcatttgtgaaattggagatgttttcaaggccaaaaacctaattgaggtaatgcggaaatctcatgaagcccgtgaaaaattgctccgtcttggaatttttagacaagtggatgttttgattgacacatgtcaaggtgatgacgcacttccaaatgggttagacgttacctttgaagtaactgaattgaggagattaacgggcagttataacaccatggttggaaacaatgaaggcagtatggtacttggcctcaagcttcctaatcttcttggtcgtgcagaaaaggtgacctttcagttttcctatggaacaaaagaaacttcgtatggcctgtccttcttcaaaccacggcccggaaacttcgaaagaaatttctctgtaaacttatataaagttactggacagttcccttggagctcactgcgggagacggacagaggaatgtcagctgagtacagttttcccatatggaagaccagccacactgtcaagtgggaaggcgtatggcgagaactgggctgcctctcaaggacggcgtcatttgctgttcgaaaagaaagcggacattcactgaaatcatctctttcgcacgccatggtcatcgattctcggaattcttccatcttaccaaggagaggtgctttgctgaaagttaaccaggaactggcaggctacactggcggggatgtgagcttcatcaaagaagattttgaacttcagttgaacaagcaactcatatttgattcagttttttcagcgtctttctggggcggaatgttggtacccattggtgataagccgtcaagcattgctgataggttttaccttgggggacccacaagcatccgcggattcagcatgcacagcatcgggccacagagcgaaggagactacctaggtggagaagcgtactgggccggcggcctgcacctctacaccccattacctttccggccaggccagggtggctttggagaacttttccgaacacacttctttctcaacgcaggaaacctctgcaacctcaactatggggagggccccaaagctcatattcgtaagctggctgagtgcatccgctggtcgtacggggccgggattgtcctcaggcttggcaacatcgctcggttggaacttaattactgcgtccccatgggagtacagacaggcgacaggatatgtgatggcgtccagtttggagctgggataaggttcctgtagccgacacccctacaggagaagctctgggactggggcagcagcaaggcgcccatgccacacaccgtctctcgaggaaacgcggttcagcgattctttgactgcggaccctgtgggaaaccccgtcaataaatgttaaagacacactccgaaaaaaaaaaaaaaaaaa

SEQ ID NO: 40 - protein, 469 aa, Homo sapiens
MGTVHARSLEPLPSSGPDFGGLGEEAEFVEVEPEAKQEILENKDVVVQHVHFDGLGRTKDDIIICEIGDVFKAKNLIEVMRKSHEAREKLLRLGIFRQVDVLIDTCQGDDALPNGLDVTFEVTELRRLTGSYNTMVGNNEGSMVLGLKLPNLLGRAEKVTFQFSYGTKETSYGLSFFKPRPGNFERNFSVNLYKVTGQFPWSSLRETDRGMSAEYSFPIWKTSHTVKWEGVWRELGCLSRTASFAVRKESGHSLKSSLSHAMVIDSRNSSILPRRGALLKVNQELAGYTGGDVSFIKEDFELQLNKQLIFDSVFSASFWGGMLVPIGDKPSSIADRFYLGGPTSIRGFSMHSIGPQSEGDYLGGEAYWAGGLHLYTPLPFRPGQGGFGELFRTHFFLNAGNLCNLNYGEGPKAHIRKLAECIRWSYGAGIVLRLGNIARLELNYCVPMGVQTGDRICDGVQFGAGIRFL

SEQ ID NO: 41 - DNA, 3018 bp, Homo sapiens
aattctctttaagagtcacagctgtccattttccacgtgcggctgaagaatggatttcagagcgctctccctccggcagtgttcacctagtaaccccttccggataaggacctgcagcccgggcgcgacccggaaagggaatccgcccttttcgcctccttcgcgccaatcgcctggagttggcgtttccgcagccgggacacagcccaccctctaagagccgcggagtcggggacggtagaaggggccgcgcgtgcgcagtggcgtccgctgtgcttccggtgcgccgggcgcggacgcgggcacgcacacacgcaagcacgcctccacttaactcgcgccgccgcggcagctcgagtccaccagcagcgccgtccgcttgaccgagatgctgcgggcctgtcagttatcgggtgtgaccgccgccgcccagagttgtctctgtgggaagtttgtcctccgtccattgcgaccatgccgcagatactctacttcaggcagctctgggttgactactggcaaaattgctggagctggccttttgtttgttggtggaggtattggtggcactatcctatatgccaaatgggattcccatttccgggaaagtgtagagaaaaccataccttactcagacaaactcttcgagatggttcttggtcctgcagcttataatgttccattgccaaagaaatcgattcagtcgggtccactaaaaatctctagtgtatcagaagtaatgaaagaatctaaacagcctgcctcacaactccaaaaacaaaagggagatactccagcttcagcaacagcacctacagaagcggctcaaattatttctgcagcaggtgataccctgtcggtcccagcccctgcagttcagcctgaggaatctttaaaaactgatcaccctgaaattggtgaaggaaaacccacacctgcactttcagaagaagcatcctcatcttctataagggagcgaccacctgaagaagttgcagctcgccttgcacaacaggaaaaacaagaacaagttaaaattgagtctctagccaagagcttagaagatgctctgaggcaaactgcaagtgtcactctgcaggctattgcagctcagaatgctgcggtccaggctgtcaatgcacactccaacatattgaaagccgccatggacaattctgagattgcaggcgagaagaaatctgctcagtggcgcacagtggagggtgcattgaaggaacgcagaaaggcagtagatgaagctgccgatgcccttctcaaagccaaagaagagttagagaagatgaaaagtgtgattgaaaatgcaaagaaaaaagaggttgctggggccaagcctcatataactgctgcagagggtaaacttcacaacatgatagttgatctggataatgtggtcaaaaaggtccaagcagctcagtctgaggctaaggttgtatctcagtatcatgagctggtggtccaagctcgggatgactttaaacgagagctggacagtattactccagaagtccttcctgggtggaaaggaatgagtgtttcagacttagctgacaagctctctactgatgatctgaactccctcattgctcatgcacatcgtcgtattgatcagctgaacagagagctggcagaacagaaggccaccgaaaagcagcacatcacgttagccttggagaaacaaaagctggaagaaaagcgggcatttgactctgcagtagcaaaagcattagaacatcacagaagtgaaatacaggctgaacaggacagaaagatagaagaagtcagagatgccatggaaaatgaaatgagaacccagcttcgccgacaggcagctgcccacactgatcacttgcgagatgtccttagggtacaagaacaggaattgaagtctgaatttgagcagaacctgtctgagaaactctctgaacaagaattacaatttcgtcgtctcagtcaagagcaagttgacaactttactctggatataaatactgcctatgccagactcagaggaatcgaacaggctgttcagagccatgcagttgctgaagaggaagccagaaaagcccaccaactctggctttcagtggaggcattaaagtacagcatgaagacctcatctgcagaaacacctactatcccgctgggtagtgcagttgaggccatcaaagccaactgttctgataatgaattcacccaagctttaaccgcagctatccctccagagtccctgacccgtggggtgtacagtgaagagacccttagagcccgtttctatgctgttcaaaaactggcccgaagggtagcaatgattgatgaaaccagaaatagcttgtaccagtacttcctctcctacctacagtccctgctcctattcccacctcagcaactgaagccgcccccagagctctgccctgaggatataaacacatttaaattactgtcatatgcttcctattgcattgagcatggtgatctggagctagcagcaaagtttgtcaatcagctgaagggggaatccagacgagtggcacaggactggctgaaggaagcccgaatgaccctagaaacgaaacagatagtggaaatcctgacagcatatgccagcgccgtaggaataggaaccactcaggtgcagccagagtgaggtttaggaagattttcataaagtcatatttcatgtcaaaggaaatcagcagtgatagatgaagggttcgcagcgagagtcccggacttgtctagaaatgagcaggtttacaagtactgttctaaatgttaacacctgttgcatttatattctttccatttgctatcatgtcagtgaacgccaggagtgctttctttgcaacttgtgtaacattttctgttttttcaggttttactgatgaggcttgtgaggccaatcaaaataatgtttgtgatctctactactgttgattttgccctcggagcaaactgaataaagcaacaagatgaaaactgaaaaaaaaaaaaaaaaaa

SEQ ID NO: 42 - protein, 758 aa, Homo sapiens
MLRACQLSGVTAAAQSCLCGKFVLRPLRPCRRYSTSGSSGLTTGKIAGAGLLFVGGGIGGTILYAKWDSHFRESVEKTIPYSDKLFEMVLGPAAYNVPLPKKSIQSGPLKISSVSEVMKESKQPASQLQKQKGDTPASATAPTEAAQIISAAGDTLSVPAPAVQPEESLKTDHPEIGEGKPTPALSEEASSSSIRERPPEEVAARLAQQEKQEQVKIESLAKSLEDALRQTASVTLQAIAAQNAAVQAVNAHSNILKAAMDNSEIAGEKKSAQWRTVEGALKERRKAVDEAADALLKAKEELEKMKSVIENAKKKEVAGAKPHITAAEGKLHNMIVDLDNVVKKVQAAQSEAKVVSQYHELVVQARDDFKRELDSITPEVLPGWKGMSVSDLADKLSTDDLNSLIAHAHRRIDQLNRELAEQKATEKQHITLALEKQKLEEKRAFDSAVAKALEHHRSEIQAEQDRKIEEVRDAMENEMRTQLRRQAAAHTDHLRDVLRVQEQELKSEFEQNLSEKLSEQELQFRRLSQEQVDNFTLDINTAYARLRGIEQAVQSHAVAEEEARKAHQLWLSVEALKYSMKTSSAETPTIPLGSAVEAIKANCSDNEFTQALTAAIPPESLTRGVYSEETLRARFYAVQKLARRVAMIDETRNSLYQYFLSYLQSLLLFPPQQLKPPPELCPEDINTFKLLSYASYCIEHGDLELAAKFVNQLKGESRRVAQDWLKEARMTLETKQIVEILTAYASAVGIGTTQVQPE

SEQ ID NO: 43 - DNA, 3015 bp, Homo sapiens
aattctctttaagagtcacagctgtccattttccacgtgcggctgaagaatggatttcagagcgctctccctccggcagtgttcacctagtaaccccttccggataaggacctgcagcccgggcgcgacccggaaagggaatccgcccttttcgcctccttcgcgccaatcgcctggagttggcgtttccgcagccgggacacagcccaccctctaagagccgcggagtcggggacggtagaaggggccgcgcgtgcgcagtggcgtccgctgtgcttccggtgcgccgggcgcggacgcgggcacgcacacacgcaagcacgcctccacttaactcgcgccgccgcggcagctcgagtccaccagcagcgccgtccgcttgaccgagatgctgcgggcctgtcagttatcgggtgtgaccgccgccgcccagagttgtctctgtgggaagtttgtcctccgtccattgcgaccatgccgcagatactctacttcaggcagctctgggttgactactggcaaaattgctggagctggccttttgtttgttggtggaggtattggtggcactatcctatatgccaaatgggattcccatttccgggaaagtgtagagaaaaccataccttactcagacaaactcttcgagatggttcttggtcctgcagcttataatgttccattgccaaagaaatcgattcagtcgggtccactaaaaatctctagtgtatcagaagtaatgaaagaatctaaacagcctgcctcacaactccaaaaacaaaagggagatactccagcttcagcaacagcacctacagaagcggctcaaattatttctgcagcaggtgataccctgtcggtcccagcccctgcagttcagcctgaggaatctttaaaaactgatcaccctgaaattggtgaaggaaaacccacacctgcactttcagaagcatcctcatcttctataagggagcgaccacctgaagaagttgcagctcgccttgcacaacaggaaaaacaagaacaagttaaaattgagtctctagccaagagcttagaagatgctctgaggcaaactgcaagtgtcactctgcaggctattgcagctcagaatgctgcggtccaggctgtcaatgcacactccaacatattgaaagccgccatggacaattctgagattgcaggcgagaagaaatctgctcagtggcgcacagtggagggtgcattgaaggaacgcagaaaggcagtagatgaagctgccgatgcccttctcaaagccaaagaagagttagagaagatgaaaagtgtgattgaaaatgcaaagaaaaaagaggttgctggggccaagcctcatataactgctgcagagggtaaacttcacaacatgatagttgatctggataatgtggtcaaaaaggtccaagcagctcagtctgaggctaaggttgtatctcagtatcatgagctggtggtccaagctcgggatgactttaaacgagagctggacagtattactccagaagtccttcctgggtggaaaggaatgagtgtttcagacttagctgacaagctctctactgatgatctgaactccctcattgctcatgcacatcgtcgtattgatcagctgaacagagagctggcagaacagaaggccaccgaaaagcagcacatcacgttagccttggagaaacaaaagctggaagaaaagcgggcatttgactctgcagtagcaaaagcattagaacatcacagaagtgaaatacaggctgaacaggacagaaagatagaagaagtcagagatgccatggaaaatgaaatgagaacccagcttcgccgacaggcagctgcccacactgatcacttgcgagatgtccttagggtacaagaacaggaattgaagtctgaatttgagcagaacctgtctgagaaactctctgaacaagaattacaatttcgtcgtctcagtcaagagcaagttgacaactttactctggatataaatactgcctatgccagactcagaggaatcgaacaggctgttcagagccatgcagttgctgaagaggaagccagaaaagcccaccaactctggctttcagtggaggcattaaagtacagcatgaagacctcatctgcagaaacacctactatcccgctgggtagtgcagttgaggccatcaaagccaactgttctgataatgaattcacccaagctttaaccgcagctatccctccagagtccctgacccgtggggtgtacagtgaagagacccttagagcccgtttctatgctgttcaaaaactggcccgaagggtagcaatgattgatgaaaccagaaatagcttgtaccagtacttcctctcctacctacagtccctgctcctattcccacctcagcaactgaagccgcccccagagctctgccctgaggatataaacacatttaaattactgtcatatgcttcctattgcattgagcatggtgatctggagctagcagcaaagtttgtcaatcagctgaagggggaatccagacgagtggcacaggactggctgaaggaagcccgaatgaccctagaaacgaaacagatagtggaaatcctgacagcatatgccagcgccgtaggaataggaaccactcaggtgcagccagagtgaggtttaggaagattttcataaagtcatatttcatgtcaaaggaaatcagcagtgatagatgaagggttcgcagcgagagtcccggacttgtctagaaatgagcaggtttacaagtactgttctaaatgttaacacctgttgcatttatattctttccatttgctatcatgtcagtgaacgccaggagtgctttctttgcaacttgtgtaacattttctgttttttcaggttttactgatgaggcttgtgaggccaatcaaaataatgtttgtgatctctactactgttgattttgccctcggagcaaactgaataaagcaacaagatgaaaactgaaaaaaaaaaaaaaaaaa

SEQ ID NO: 44 - protein, 757 aa, Homo sapiens
MLRACQLSGVTAAAQSCLCGKFVLRPLRPCRRYSTSGSSGLTTGKIAGAGLLFVGGGIGGTILYAKWDSHFRESVEKTIPYSDKLFEMVLGPAAYNVPLPKKSIQSGPLKISSVSEVMKESKQPASQLQKQKGDTPASATAPTEAAQIISAAGDTLSVPAPAVQPEESLKTDHPEIGEGKPTPALSEASSSSIRERPPEEVAARLAQQEKQEQVKIESLAKSLEDALRQTASVTLQAIAAQNAAVQAVNAHSNILKAAMDNSEIAGEKKSAQWRTVEGALKERRKAVDEAADALLKAKEELEKMKSVIENAKKKEVAGAKPHITAAEGKLHNMIVDLDNVVKKVQAAQSEAKVVSQYHELVVQARDDFKRELDSITPEVLPGWKGMSVSDLADKLSTDDLNSLIAHAHRRIDQLNRELAEQKATEKQHITLALEKQKLEEKRAFDSAVAKALEHHRSEIQAEQDRKIEEVRDAMENEMRTQLRRQAAAHTDHLRDVLRVQEQELKSEFEQNLSEKLSEQELQFRRLSQEQVDNFTLDINTAYARLRGIEQAVQSHAVAEEEARKAHQLWLSVEALKYSMKTSSAETPTIPLGSAVEAIKANCSDNEFTQALTAAIPPESLTRGVYSEETLRARFYAVQKLARRVAMIDETRNSLYQYFLSYLQSLLLFPPQQLKPPPELCPEDINTFKLLSYASYCIEHGDLELAAKFVNQLKGESRRVAQDWLKEARMTLETKQIVEILTAYASAVGIGTTQVQPE

SEQ ID NO: 45 - DNA, 2985 bp, Homo sapiens
aattctctttaagagtcacagctgtccattttccacgtgcggctgaagaatggatttcagagcgctctccctccggcagtgttcacctagtaaccccttccggataaggacctgcagcccgggcgcgacccggaaagggaatccgcccttttcgcctccttcgcgccaatcgcctggagttggcgtttccgcagccgggacacagcccaccctctaagagccgcggagtcggggacggtagaaggggccgcgcgtgcgcagtggcgtccgctgtgcttccggtgcgccgggcgcggacgcgggcacgcacacacgcaagcacgcctccacttaactcgcgccgccgcggcagctcgagtccaccagcagcgccgtccgcttgaccgagatgctgcgggcctgtcagttatcgggtgtgaccgccgccgcccagagttgtctctgtgggaagtttgtcctccgtccattgcgaccatgccgcagatactctacttcaggcagctctgggttgactactggcaaaattgctggagctggccttttgtttgttggtggaggtattggtggcactatcctatatgccaaatgggattcccatttccgggaaagtgtagagaaaaccataccttactcagacaaactcttcgagatggttcttggtcctgcagcttataatgttccattgccaaagaaatcgattcagtcgggtccactaaaaatctctagtgtatcagaagtaatgaaagaatctaaacagcctgcctcacaactccaaaaacaaaagggagatactccagcttcagcaacagcaggtgataccctgtcggtcccagcccctgcagttcagcctgaggaatctttaaaaactgatcaccctgaaattggtgaaggaaaacccacacctgcactttcagaagaagcatcctcatcttctataagggagcgaccacctgaagaagttgcagctcgccttgcacaacaggaaaaacaagaacaagttaaaattgagtctctagccaagagcttagaagatgctctgaggcaaactgcaagtgtcactctgcaggctattgcagctcagaatgctgcggtccaggctgtcaatgcacactccaacatattgaaagccgccatggacaattctgagattgcaggcgagaagaaatctgctcagtggcgcacagtggagggtgcattgaaggaacgcagaaaggcagtagatgaagctgccgatgcccttctcaaagccaaagaagagttagagaagatgaaaagtgtgattgaaaatgcaaagaaaaaagaggttgctggggccaagcctcatataactgctgcagagggtaaacttcacaacatgatagttgatctggataatgtggtcaaaaaggtccaagcagctcagtctgaggctaaggttgtatctcagtatcatgagctggtggtccaagctcgggatgactttaaacgagagctggacagtattactccagaagtccttcctgggtggaaaggaatgagtgtttcagacttagctgacaagctctctactgatgatctgaactccctcattgctcatgcacatcgtcgtattgatcagctgaacagagagctggcagaacagaaggccaccgaaaagcagcacatcacgttagccttggagaaacaaaagctggaagaaaagcgggcatttgactctgcagtagcaaaagcattagaacatcacagaagtgaaatacaggctgaacaggacagaaagatagaagaagtcagagatgccatggaaaatgaaatgagaacccagcttcgccgacaggcagctgcccacactgatcacttgcgagatgtccttagggtacaagaacaggaattgaagtctgaatttgagcagaacctgtctgagaaactctctgaacaagaattacaatttcgtcgtctcagtcaagagcaagttgacaactttactctggatataaatactgcctatgccagactcagaggaatcgaacaggctgttcagagccatgcagttgctgaagaggaagccagaaaagcccaccaactctggctttcagtggaggcattaaagtacagcatgaagacctcatctgcagaaacacctactatcccgctgggtagtgcagttgaggccatcaaagccaactgttctgataatgaattcacccaagctttaaccgcagctatccctccagagtccctgacccgtggggtgtacagtgaagagacccttagagcccgtttctatgctgttcaaaaactggcccgaagggtagcaatgattgatgaaaccagaaatagcttgtaccagtacttcctctcctacctacagtccctgctcctattcccacctcagcaactgaagccgcccccagagctctgccctgaggatataaacacatttaaattactgtcatatgcttcctattgcattgagcatggtgatctggagctagcagcaaagtttgtcaatcagctgaagggggaatccagacgagtggcacaggactggctgaaggaagcccgaatgaccctagaaacgaaacagatagtggaaatcctgacagcatatgccagcgccgtaggaataggaaccactcaggtgcagccagagtgaggtttaggaagattttcataaagtcatatttcatgtcaaaggaaatcagcagtgatagatgaagggttcgcagcgagagtcccggacttgtctagaaatgagcaggtttacaagtactgttctaaatgttaacacctgttgcatttatattctttccatttgctatcatgtcagtgaacgccaggagtgctttctttgcaacttgtgtaacattttctgttttttcaggttttactgatgaggcttgtgaggccaatcaaaataatgtttgtgatctctactactgttgattttgccctcggagcaaactgaataaagcaacaagatgaaaactgaaaaaaaaaaaaaaaaaa

SEQ ID NO: 46 - protein, 747 aa, Homo sapiens
MLRACQLSGVTAAAQSCLCGKFVLRPLRPCRRYSTSGSSGLTTGKIAGAGLLFVGGGIGGTILYAKWDSHFRESVEKTIPYSDKLFEMVLGPAAYNVPLPKKSIQSGPLKISSVSEVMKESKQPASQLQKQKGDTPASATAGDTLSVPAPAVQPEESLKTDHPEIGEGKPTPALSEEASSSSIRERPPEEVAARLAQQEKQEQVKIESLAKSLEDALRQTASVTLQAIAAQNAAVQAVNAHSNILKAAMDNSEIAGEKKSAQWRTVEGALKERRKAVDEAADALLKAKEELEKMKSVIENAKKKEVAGAKPHITAAEGKLHNMIVDLDNVVKKVQAAQSEAKVVSQYHELVVQARDDFKRELDSITPEVLPGWKGMSVSDLADKLSTDDLNSLIAHAHRRIDQLNRELAEQKATEKQHITLALEKQKLEEKRAFDSAVAKALEHHRSEIQAEQDRKIEEVRDAMENEMRTQLRRQAAAHTDHLRDVLRVQEQELKSEFEQNLSEKLSEQELQFRRLSQEQVDNFTLDINTAYARLRGIEQAVQSHAVAEEEARKAHQLWLSVEALKYSMKTSSAETPTIPLGSAVEAIKANCSDNEFTQALTAAIPPESLTRGVYSEETLRARFYAVQKLARRVAMIDETRNSLYQYFLSYLQSLLLFPPQQLKPPPELCPEDINTFKLLSYASYCIEHGDLELAAKFVNQLKGESRRVAQDWLKEARMTLETKQIVEILTAYASAVGIGTTQVQPE

SEQ ID NO: 47 - protein, 15 aa, Homo sapiens
YLILGSAVGGGYTAK

SEQ ID NO: 48 - protein, 6 aa, Homo sapiens
TFDQWK

SEQ ID NO: 49 - protein, 10 aa, Homo sapiens
DMIPDLSEYK

SEQ ID NO: 50 - protein, 18 aa, Homo sapiens
WIVPDIVWEIDEYIDFEK

SEQ ID NO: 51 - protein, 7 aa, Homo sapiens
LAPDFDK

SEQ ID NO: 52 - protein, 9 aa, Homo sapiens
IVESLSLLK

SEQ ID NO: 53 - protein, 10 aa, Homo sapiens
ALPNSEDLVK

SEQ ID NO: 54 - protein, 14 aa, Homo sapiens
DFFTSGSPEETAFR

SEQ ID NO: 55 - protein, 13 aa, Homo sapiens
TRLLKLRYLILGS

SEQ ID NO: 56 - protein, 20 aa, Homo sapiens
FWPARLATRLLKLRYLILGS

SEQ ID NO: 57 - protein, 21 aa, Homo sapiens
GLLGELILLQQQIQEHEEEAR

SEQ ID NO: 58 - protein, 13 aa, Homo sapiens
AAGQYSTSYAQQK

SEQ ID NO: 59 - protein, 14 aa, Homo sapiens
IDQLQEELLHTQLK

SEQ ID NO: 60 - protein, 37 aa, Homo sapiens
EYKWIVPDIVWEIDEYIDFGHKLVSEVIGASDLLLLL

SEQ ID NO: 61 - protein, 42 aa, Homo sapiens
EYKWIVPDIVWEIDEYIDFGSPEETAFRATDRGSESDKHFRK

SEQ ID NO: 62 - protein, 59 aa, Homo sapiens
EKIRKALPNSEDLVKLAPDFDKIVESLSLLKDFFTSGSPEETAFRATDRGSESDKHFRK

SEQ ID NO: 63 - protein, 60 aa, Homo sapiens
GSPEETAFRATDRGSESDKHFRKVSDKEKIDQLQEELLHTQLKYQRILERLEKENKELRK